European Patent Application EP 4 144 840 A1, published March 8, 2023. Title: PARENT PHYTASE VARIANT. Applicant: NANJING BESTZYME BIO-ENGINEERING CO., LTD. The sequence listing filed with the application follows.

SEQUENCE LISTING (118 sequences)

SEQ ID NO: 1 - protein, 410 aa, Escherichia coli
QSEPELKLESVVIVSRHGVRAPTKATQLMQDVTPDAWPTWPVKLGWLTPRGGELIAYLGHYQRQRLVADGLLAKKGCPQSGQVAIIADVDERTRKTGEAFAAGLAPDCAITVHTQADTSSPDPLFNPLKTGVCQLDNANVTDAILSRAGGSIADFTGHRQTAFRELERVLNFPQSNLCLKREKQDESCSLTQALPSELKVSADNVSLTGAVSLASMLTKIFLLQQAQGMPEPGWGRITDSHQWNTLLSLHNAQFYLLQRTPEVARSRATPLLDLIKTALTPHPPQKQAYGVTLPTSVLFIAGHDTNLANLGGALELNWTLPGQPDNTPPGGELVFERWRRLSDNSQWIQVSLVFQTLQQMRDKTPLSLNTPPGEVKLTLAGCEERNAQGMCSLAGFTQIVNEARIPACSL

SEQ ID NO: 2 - protein, 410 aa, Artificial Sequence
  APPA-Y0
QSEPELKLESVVIVSRHGVRAPTKATQLMQDVTPDAWPTWPVKLGELTPRGGELIAYLGHYWRQRLVADELLPNQTCPQSGQVAIIADVDERTRKTGEAFAAGLAPDCAITVHTQADTSSPDPLFNPLKTGVCQLDNANVTDAILERAGGSIADFTGHYQTAFRELERVLNFSQSNLCLKREKQDESCSLTQALPSELKVSADNVSLTGAVSLASMLTEIFLLQQAQGMPEPGWGRITDSHQWNTLLSLHNAQFDLLQRTPEVARSRATPLLDLIKTALTPNGTQKQAYGVTLPTSVLFIAGHDTNLANLGGALELNWTLPGQPDNTPPGGELVFERWRRLSDNSCWIQVSLVFQTLQQMRDKTPLSLNTPPGEVKLTLAGCEERNAQGMCSCAGFTQIVNEARIPACSL

SEQ ID NO: 3 - protein, 410 aa, Artificial Sequence
  APPA-Y1
QSEPELKLESVVIVSRHGVRAPTKPTQLMQDVTPDAWPTWPVKLGELTPRGGELIAYLGHYWRQRLVADELLPNQTCPQSGQVAIIADVDERTRKTGEAFAAGLAPDCAITVHTQADTSSPDPLFNPLKTGVCQLDNANVTDAILERAGGSIADFTGHYQTAFRELERVLNFSQSNLCLKREKQDESCSLTQALPSELKVSADNVSLTGAVSLASMLTEIFLLQQAQGMPEPGWGRITDSHQWNTLLSLHNAQFDLLQRTPEVARSRATPLLDLIKTALTPNGTQKQAYGVTLPTSVLFIAGHDTNLANLGGALELNWTLPGQPDNTPPGGELVFERWRRLSDNSCWIQVSLVFQTLQQMRDKTPLSLNTPPGEVKLTLAGCEERNAQGMCSCAGFTQIVNEARIPACSL

SEQ ID NO: 4 - protein, 410 aa, Artificial Sequence
  APPA-Y2
QSEPELKLESVVIVSRHGVRAPTKATQLLQDVTPDAWPTWPVKLGELTPRGGELIAYLGHYWRQRLVADELLPNQTCPQSGQVAIIADVDERTRKTGEAFAAGLAPDCAITVHTQADTSSPDPLFNPLKTGVCQLDNANVTDAILERAGGSIADFTGHYQTAFRELERVLNFSQSNLCLKREKQDESCSLTQALPSELKVSADNVSLTGAVSLASMLTEIFLLQQAQGMPEPGWGRITDSHQWNTLLSLHNAQFDLLQRTPEVARSRATPLLDLIKTALTPNGTQKQAYGVTLPTSVLFIAGHDTNLANLGGALELNWTLPGQPDNTPPGGELVFERWRRLSDNSCWIQVSLVFQTLQQMRDKTPLSLNTPPGEVKLTLAGCEERNAQGMCSCAGFTQIVNEARIPACSL

SEQ ID NO: 5 - protein, 410 aa, Artificial Sequence
  APPA-Y3
QSEPELKLESVVIVSRHGVRAPTKATQLMQDVTPDAWPTWPVPLGELTPRGGELIAYLGHYWRQRLVADELLPNQTCPQSGQVAIIADVDERTRKTGEAFAAGLAPDCAITVHTQADTSSPDPLFNPLKTGVCQLDNANVTDAILERAGGSIADFTGHYQTAFRELERVLNFSQSNLCLKREKQDESCSLTQALPSELKVSADNVSLTGAVSLASMLTEIFLLQQAQGMPEPGWGRITDSHQWNTLLSLHNAQFDLLQRTPEVARSRATPLLDLIKTALTPNGTQKQAYGVTLPTSVLFIAGHDTNLANLGGALELNWTLPGQPDNTPPGGELVFERWRRLSDNSCWIQVSLVFQTLQQMRDKTPLSLNTPPGEVKLTLAGCEERNAQGMCSCAGFTQIVNEARIPACSL

SEQ ID NO: 6 - protein, 410 aa, Artificial Sequence
  APPA-Y4
QSEPELKLESVVIVSRHGVRAPTKATQLMQDVTPDAWPTWPVKLGELTPKGGELIAYLGHYWRQRLVADELLPNQTCPQSGQVAIIADVDERTRKTGEAFAAGLAPDCAITVHTQADTSSPDPLFNPLKTGVCQLDNANVTDAILERAGGSIADFTGHYQTAFRELERVLNFSQSNLCLKREKQDESCSLTQALPSELKVSADNVSLTGAVSLASMLTEIFLLQQAQGMPEPGWGRITDSHQWNTLLSLHNAQFDLLQRTPEVARSRATPLLDLIKTALTPNGTQKQAYGVTLPTSVLFIAGHDTNLANLGGALELNWTLPGQPDNTPPGGELVFERWRRLSDNSCWIQVSLVFQTLQQMRDKTPLSLNTPPGEVKLTLAGCEERNAQGMCSCAGFTQIVNEARIPACSL

SEQ ID NO: 7 - protein, 410 aa, Artificial Sequence
  APPA-Y5
QSEPELKLESVVIVSRHGVRAPTKATQLMQDVTPDAWPTWPVKLGELTPRGAELIAYLGHYWRQRLVADELLPNQTCPQSGQVAIIADVDERTRKTGEAFAAGLAPDCAITVHTQADTSSPDPLFNPLKTGVCQLDNANVTDAILERAGGSIADFTGHYQTAFRELERVLNFSQSNLCLKREKQDESCSLTQALPSELKVSADNVSLTGAVSLASMLTEIFLLQQAQGMPEPGWGRITDSHQWNTLLSLHNAQFDLLQRTPEVARSRATPLLDLIKTALTPNGTQKQAYGVTLPTSVLFIAGHDTNLANLGGALELNWTLPGQPDNTPPGGELVFERWRRLSDNSCWIQVSLVFQTLQQMRDKTPLSLNTPPGEVKLTLAGCEERNAQGMCSCAGFTQIVNEARIPACSL

SEQ ID NO: 8 - protein, 410 aa, Artificial Sequence
  APPA-Y6
QSEPELKLESVVIVSRHGVRAPTKATQLMQDVTPDAWPTWPVKLGELTPRGGELIAYMGHYWRQRLVADELLPNQTCPQSGQVAIIADVDERTRKTGEAFAAGLAPDCAITVHTQADTSSPDPLFNPLKTGVCQLDNANVTDAILERAGGSIADFTGHYQTAFRELERVLNFSQSNLCLKREKQDESCSLTQALPSELKVSADNVSLTGAVSLASMLTEIFLLQQAQGMPEPGWGRITDSHQWNTLLSLHNAQFDLLQRTPEVARSRATPLLDLIKTALTPNGTQKQAYGVTLPTSVLFIAGHDTNLANLGGALELNWTLPGQPDNTPPGGELVFERWRRLSDNSCWIQVSLVFQTLQQMRDKTPLSLNTPPGEVKLTLAGCEERNAQGMCSCAGFTQIVNEARIPACSL

SEQ ID NO: 9 - protein, 410 aa, Artificial Sequence
  APPA-Y7
QSEPELKLESVVIVSRHGVRAPTKATQLMQDVTPDAWPTWPVKLGELTPRGGELIAYLGHYWRQRLVAQELLPNQTCPQSGQVAIIADVDERTRKTGEAFAAGLAPDCAITVHTQADTSSPDPLFNPLKTGVCQLDNANVTDAILERAGGSIADFTGHYQTAFRELERVLNFSQSNLCLKREKQDESCSLTQALPSELKVSADNVSLTGAVSLASMLTEIFLLQQAQGMPEPGWGRITDSHQWNTLLSLHNAQFDLLQRTPEVARSRATPLLDLIKTALTPNGTQKQAYGVTLPTSVLFIAGHDTNLANLGGALELNWTLPGQPDNTPPGGELVFERWRRLSDNSCWIQVSLVFQTLQQMRDKTPLSLNTPPGEVKLTLAGCEERNAQGMCSCAGFTQIVNEARIPACSL

SEQ ID NO: 10 - protein, 410 aa, Artificial Sequence
  APPA-Y8
QSEPELKLESVVIVSRHGVRAPTKATQLMQDVTPDAWPTWPVKLGELTPRGGELIAYLGHYWRQRLVADELLPNQTCPQSGQVAIIADVDERTRKTAEAFAAGLAPDCAITVHTQADTSSPDPLFNPLKTGVCQLDNANVTDAILERAGGSIADFTGHYQTAFRELERVLNFSQSNLCLKREKQDESCSLTQALPSELKVSADNVSLTGAVSLASMLTEIFLLQQAQGMPEPGWGRITDSHQWNTLLSLHNAQFDLLQRTPEVARSRATPLLDLIKTALTPNGTQKQAYGVTLPTSVLFIAGHDTNLANLGGALELNWTLPGQPDNTPPGGELVFERWRRLSDNSCWIQVSLVFQTLQQMRDKTPLSLNTPPGEVKLTLAGCEERNAQGMCSCAGFTQIVNEARIPACSL

SEQ ID NO: 11 - protein, 410 aa, Artificial Sequence
  APPA-Y9
QSEPELKLESVVIVSRHGVRAPTKATQLMQDVTPDAWPTWPVKLGELTPRGGELIAYLGHYWRQRLVADELLPNQTCPQSGQVAIIADVDERTRKTGQAFAAGLAPDCAITVHTQADTSSPDPLFNPLKTGVCQLDNANVTDAILERAGGSIADFTGHYQTAFRELERVLNFSQSNLCLKREKQDESCSLTQALPSELKVSADNVSLTGAVSLASMLTEIFLLQQAQGMPEPGWGRITDSHQWNTLLSLHNAQFDLLQRTPEVARSRATPLLDLIKTALTPNGTQKQAYGVTLPTSVLFIAGHDTNLANLGGALELNWTLPGQPDNTPPGGELVFERWRRLSDNSCWIQVSLVFQTLQQMRDKTPLSLNTPPGEVKLTLAGCEERNAQGMCSCAGFTQIVNEARIPACSL

SEQ ID NO: 12 - protein, 410 aa, Artificial Sequence
  APPA-Y10
QSEPELKLESVVIVSRHGVRAPTKATQLMQDVTPDAWPTWPVKLGELTPRGGELIAYLGHYWRQRLVADELLPNQTCPQSGQVAIIADVDERTRKTGEAFAAGLFPDCAITVHTQADTSSPDPLFNPLKTGVCQLDNANVTDAILERAGGSIADFTGHYQTAFRELERVLNFSQSNLCLKREKQDESCSLTQALPSELKVSADNVSLTGAVSLASMLTEIFLLQQAQGMPEPGWGRITDSHQWNTLLSLHNAQFDLLQRTPEVARSRATPLLDLIKTALTPNGTQKQAYGVTLPTSVLFIAGHDTNLANLGGALELNWTLPGQPDNTPPGGELVFERWRRLSDNSCWIQVSLVFQTLQQMRDKTPLSLNTPPGEVKLTLAGCEERNAQGMCSCAGFTQIVNEARIPACSL

SEQ ID NO: 13 - protein, 410 aa, Artificial Sequence
  APPA-Y11
QSEPELKLESVVIVSRHGVRAPTKATQLMQDVTPDAWPTWPVKLGELTPRGGELIAYLGHYWRQRLVADELLPNQTCPQSGQVAIIADVDERTRKTGEAFAAGLAPDCDITVHTQADTSSPDPLFNPLKTGVCQLDNANVTDAILERAGGSIADFTGHYQTAFRELERVLNFSQSNLCLKREKQDESCSLTQALPSELKVSADNVSLTGAVSLASMLTEIFLLQQAQGMPEPGWGRITDSHQWNTLLSLHNAQFDLLQRTPEVARSRATPLLDLIKTALTPNGTQKQAYGVTLPTSVLFIAGHDTNLANLGGALELNWTLPGQPDNTPPGGELVFERWRRLSDNSCWIQVSLVFQTLQQMRDKTPLSLNTPPGEVKLTLAGCEERNAQGMCSCAGFTQIVNEARIPACSL

SEQ ID NO: 14 - protein, 410 aa, Artificial Sequence
  APPA-Y12
QSEPELKLESVVIVSRHGVRAPTKATQLMQDVTPDAWPTWPVKLGELTPRGGELIAYLGHYWRQRLVADELLPNQTCPQSGQVAIIADVDERTRKTGEAFAAGLAPDCAITVHTQADQSSPDPLFNPLKTGVCQLDNANVTDAILERAGGSIADFTGHYQTAFRELERVLNFSQSNLCLKREKQDESCSLTQALPSELKVSADNVSLTGAVSLASMLTEIFLLQQAQGMPEPGWGRITDSHQWNTLLSLHNAQFDLLQRTPEVARSRATPLLDLIKTALTPNGTQKQAYGVTLPTSVLFIAGHDTNLANLGGALELNWTLPGQPDNTPPGGELVFERWRRLSDNSCWIQVSLVFQTLQQMRDKTPLSLNTPPGEVKLTLAGCEERNAQGMCSCAGFTQIVNEARIPACSL

SEQ ID NO: 15 - protein, 410 aa, Artificial Sequence
  APPA-Y13
QSEPELKLESVVIVSRHGVRAPTKATQLMQDVTPDAWPTWPVKLGELTPRGGELIAYLGHYWRQRLVADELLPNQTCPQSGQVAIIADVDERTRKTGEAFAAGLAPDCAITVHTQADTSTPDPLFNPLKTGVCQLDNANVTDAILERAGGSIADFTGHYQTAFRELERVLNFSQSNLCLKREKQDESCSLTQALPSELKVSADNVSLTGAVSLASMLTEIFLLQQAQGMPEPGWGRITDSHQWNTLLSLHNAQFDLLQRTPEVARSRATPLLDLIKTALTPNGTQKQAYGVTLPTSVLFIAGHDTNLANLGGALELNWTLPGQPDNTPPGGELVFERWRRLSDNSCWIQVSLVFQTLQQMRDKTPLSLNTPPGEVKLTLAGCEERNAQGMCSCAGFTQIVNEARIPACSL

SEQ ID NO: 16 - protein, 410 aa, Artificial Sequence
  APPA-Y14
QSEPELKLESVVIVSRHGVRAPTKATQLMQDVTPDAWPTWPVKLGELTPRGGELIAYLGHYWRQRLVADELLPNQTCPQSGQVAIIADVDERTRKTGEAFAAGLAPDCAITVHTQADTSSMDPLFNPLKTGVCQLDNANVTDAILERAGGSIADFTGHYQTAFRELERVLNFSQSNLCLKREKQDESCSLTQALPSELKVSADNVSLTGAVSLASMLTEIFLLQQAQGMPEPGWGRITDSHQWNTLLSLHNAQFDLLQRTPEVARSRATPLLDLIKTALTPNGTQKQAYGVTLPTSVLFIAGHDTNLANLGGALELNWTLPGQPDNTPPGGELVFERWRRLSDNSCWIQVSLVFQTLQQMRDKTPLSLNTPPGEVKLTLAGCEERNAQGMCSCAGFTQIVNEARIPACSL

SEQ ID NO: 17 - protein, 410 aa, Artificial Sequence
  APPA-Y15
QSEPELKLESVVIVSRHGVRAPTKATQLMQDVTPDAWPTWPVKLGELTPRGGELIAYLGHYWRQRLVADELLPNQTCPQSGQVAIIADVDERTRKTGEAFAAGLAPDCAITVHTQADTSSPDPLFNPLKTGVCQLDIANVTDAILERAGGSIADFTGHYQTAFRELERVLNFSQSNLCLKREKQDESCSLTQALPSELKVSADNVSLTGAVSLASMLTEIFLLQQAQGMPEPGWGRITDSHQWNTLLSLHNAQFDLLQRTPEVARSRATPLLDLIKTALTPNGTQKQAYGVTLPTSVLFIAGHDTNLANLGGALELNWTLPGQPDNTPPGGELVFERWRRLSDNSCWIQVSLVFQTLQQMRDKTPLSLNTPPGEVKLTLAGCEERNAQGMCSCAGFTQIVNEARIPACSL

SEQ ID NO: 18 - protein, 410 aa, Artificial Sequence
  APPA-Y16
QSEPELKLESVVIVSRHGVRAPTKATQLMQDVTPDAWPTWPVKLGELTPRGGELIAYLGHYWRQRLVADELLPNQTCPQSGQVAIIADVDERTRKTGEAFAAGLAPDCAITVHTQADTSSPDPLFNPLKTGVCQLDNANVTDAILERAGGSIADFMGHYQTAFRELERVLNFSQSNLCLKREKQDESCSLTQALPSELKVSADNVSLTGAVSLASMLTEIFLLQQAQGMPEPGWGRITDSHQWNTLLSLHNAQFDLLQRTPEVARSRATPLLDLIKTALTPNGTQKQAYGVTLPTSVLFIAGHDTNLANLGGALELNWTLPGQPDNTPPGGELVFERWRRLSDNSCWIQVSLVFQTLQQMRDKTPLSLNTPPGEVKLTLAGCEERNAQGMCSCAGFTQIVNEARIPACSL

SEQ ID NO: 19 - protein, 410 aa, Artificial Sequence
  APPA-Y17
QSEPELKLESVVIVSRHGVRAPTKATQLMQDVTPDAWPTWPVKLGELTPRGGELIAYLGHYWRQRLVADELLPNQTCPQSGQVAIIADVDERTRKTGEAFAAGLAPDCAITVHTQADTSSPDPLFNPLKTGVCQLDNANVTDAILERAGGSIADFTGHLQTAFRELERVLNFSQSNLCLKREKQDESCSLTQALPSELKVSADNVSLTGAVSLASMLTEIFLLQQAQGMPEPGWGRITDSHQWNTLLSLHNAQFDLLQRTPEVARSRATPLLDLIKTALTPNGTQKQAYGVTLPTSVLFIAGHDTNLANLGGALELNWTLPGQPDNTPPGGELVFERWRRLSDNSCWIQVSLVFQTLQQMRDKTPLSLNTPPGEVKLTLAGCEERNAQGMCSCAGFTQIVNEARIPACSL

SEQ ID NO: 20 - protein, 410 aa, Artificial Sequence
  APPA-Y18
QSEPELKLESVVIVSRHGVRAPTKATQLMQDVTPDAWPTWPVKLGELTPRGGELIAYLGHYWRQRLVADELLPNQTCPQSGQVAIIADVDERTRKTGEAFAAGLAPDCAITVHTQADTSSPDPLFNPLKTGVCQLDNANVTDAILERAGGSIADFTGHYQTAFRELERVLNFSQSNLCLKREKQDESCSLPQALPSELKVSADNVSLTGAVSLASMLTEIFLLQQAQGMPEPGWGRITDSHQWNTLLSLHNAQFDLLQRTPEVARSRATPLLDLIKTALTPNGTQKQAYGVTLPTSVLFIAGHDTNLANLGGALELNWTLPGQPDNTPPGGELVFERWRRLSDNSCWIQVSLVFQTLQQMRDKTPLSLNTPPGEVKLTLAGCEERNAQGMCSCAGFTQIVNEARIPACSL

SEQ ID NO: 21 - protein, 410 aa, Artificial Sequence
  APPA-Y19
QSEPELKLESVVIVSRHGVRAPTKATQLMQDVTPDAWPTWPVKLGELTPRGGELIAYLGHYWRQRLVADELLPNQTCPQSGQVAIIADVDERTRKTGEAFAAGLAPDCAITVHTQADTSSPDPLFNPLKTGVCQLDNANVTDAILERAGGSIADFTGHYQTAFRELERVLNFSQSNLCLKREKQDESCSLTQALPSELKVSADNVSLTGALSLASMLTEIFLLQQAQGMPEPGWGRITDSHQWNTLLSLHNAQFDLLQRTPEVARSRATPLLDLIKTALTPNGTQKQAYGVTLPTSVLFIAGHDTNLANLGGALELNWTLPGQPDNTPPGGELVFERWRRLSDNSCWIQVSLVFQTLQQMRDKTPLSLNTPPGEVKLTLAGCEERNAQGMCSCAGFTQIVNEARIPACSL

SEQ ID NO: 22 - protein, 410 aa, Artificial Sequence
  APPA-Y20
QSEPELKLESVVIVSRHGVRAPTKATQLMQDVTPDAWPTWPVKLGELTPRGGELIAYLGHYWRQRLVADELLPNQTCPQSGQVAIIADVDERTRKTGEAFAAGLAPDCAITVHTQADTSSPDPLFNPLKTGVCQLDNANVTDAILERAGGSIADFTGHYQTAFRELERVLNFSQSNLCLKREKQDESCSLTQALPSELKVSADNVSLTGAVSLASMLTEIFLLQYAQGMPEPGWGRITDSHQWNTLLSLHNAQFDLLQRTPEVARSRATPLLDLIKTALTPNGTQKQAYGVTLPTSVLFIAGHDTNLANLGGALELNWTLPGQPDNTPPGGELVFERWRRLSDNSCWIQVSLVFQTLQQMRDKTPLSLNTPPGEVKLTLAGCEERNAQGMCSCAGFTQIVNEARIPACSL

SEQ ID NO: 23 - protein, 410 aa, Artificial Sequence
  APPA-Y21
QSEPELKLESVVIVSRHGVRAPTKATQLMQDVTPDAWPTWPVKLGELTPRGGELIAYLGHYWRQRLVADELLPNQTCPQSGQVAIIADVDERTRKTGEAFAAGLAPDCAITVHTQADTSSPDPLFNPLKTGVCQLDNANVTDAILERAGGSIADFTGHYQTAFRELERVLNFSQSNLCLKREKQDESCSLTQALPSELKVSADNVSLTGAVSLASMLTEIFLLQQAQGMPEPGWGRITDWHQWNTLLSLHNAQFDLLQRTPEVARSRATPLLDLIKTALTPNGTQKQAYGVTLPTSVLFIAGHDTNLANLGGALELNWTLPGQPDNTPPGGELVFERWRRLSDNSCWIQVSLVFQTLQQMRDKTPLSLNTPPGEVKLTLAGCEERNAQGMCSCAGFTQIVNEARIPACSL

SEQ ID NO: 24 - protein, 410 aa, Artificial Sequence
  APPA-Y22
QSEPELKLESVVIVSRHGVRAPTKATQLMQDVTPDAWPTWPVKLGELTPRGGELIAYLGHYWRQRLVADELLPNQTCPQSGQVAIIADVDERTRKTGEAFAAGLAPDCAITVHTQADTSSPDPLFNPLKTGVCQLDNANVTDAILERAGGSIADFTGHYQTAFRELERVLNFSQSNLCLKREKQDESCSLTQALPSELKVSADNVSLTGAVSLASMLTEIFLLQQAQGMPEPGWGRITDSHQWYTLLSLHNAQFDLLQRTPEVARSRATPLLDLIKTALTPNGTQKQAYGVTLPTSVLFIAGHDTNLANLGGALELNWTLPGQPDNTPPGGELVFERWRRLSDNSCWIQVSLVFQTLQQMRDKTPLSLNTPPGEVKLTLAGCEERNAQGMCSCAGFTQIVNEARIPACSL

SEQ ID NO: 25 - protein, 410 aa, Artificial Sequence
  APPA-Y23
QSEPELKLESVVIVSRHGVRAPTKATQLMQDVTPDAWPTWPVKLGELTPRGGELIAYLGHYWRQRLVADELLPNQTCPQSGQVAIIADVDERTRKTGEAFAAGLAPDCAITVHTQADTSSPDPLFNPLKTGVCQLDNANVTDAILERAGGSIADFTGHYQTAFRELERVLNFSQSNLCLKREKQDESCSLTQALPSELKVSADNVSLTGAVSLASMLTEIFLLQQAQGMPEPGWGRITDSHQWNTLLSLHNAQFDLLFRTPEVARSRATPLLDLIKTALTPNGTQKQAYGVTLPTSVLFIAGHDTNLANLGGALELNWTLPGQPDNTPPGGELVFERWRRLSDNSCWIQVSLVFQTLQQMRDKTPLSLNTPPGEVKLTLAGCEERNAQGMCSCAGFTQIVNEARIPACSL

SEQ ID NO: 26 - protein, 410 aa, Artificial Sequence
  APPA-Y24
QSEPELKLESVVIVSRHGVRAPTKATQLMQDVTPDAWPTWPVKLGELTPRGGELIAYLGHYWRQRLVADELLPNQTCPQSGQVAIIADVDERTRKTGEAFAAGLAPDCAITVHTQADTSSPDPLFNPLKTGVCQLDNANVTDAILERAGGSIADFTGHYQTAFRELERVLNFSQSNLCLKREKQDESCSLTQALPSELKVSADNVSLTGAVSLASMLTEIFLLQQAQGMPEPGWGRITDSHQWNTLLSLHNAQFDLLQRTPEVARYRATPLLDLIKTALTPNGTQKQAYGVTLPTSVLFIAGHDTNLANLGGALELNWTLPGQPDNTPPGGELVFERWRRLSDNSCWIQVSLVFQTLQQMRDKTPLSLNTPPGEVKLTLAGCEERNAQGMCSCAGFTQIVNEARIPACSL

SEQ ID NO: 27 - protein, 410 aa, Artificial Sequence
  APPA-Y25
QSEPELKLESVVIVSRHGVRAPTKATQLMQDVTPDAWPTWPVKLGELTPRGGELIAYLGHYWRQRLVADELLPNQTCPQSGQVAIIADVDERTRKTGEAFAAGLAPDCAITVHTQADTSSPDPLFNPLKTGVCQLDNANVTDAILERAGGSIADFTGHYQTAFRELERVLNFSQSNLCLKREKQDESCSLTQALPSELKVSADNVSLTGAVSLASMLTEIFLLQQAQGMPEPGWGRITDSHQWNTLLSLHNAQFDLLQRTPEVARSRATPLLDLIKTALTPNGTQKQAYGVTLPPSVLFIAGHDTNLANLGGALELNWTLPGQPDNTPPGGELVFERWRRLSDNSCWIQVSLVFQTLQQMRDKTPLSLNTPPGEVKLTLAGCEERNAQGMCSCAGFTQIVNEARIPACSL

SEQ ID NO: 28 - protein, 410 aa, Artificial Sequence
  APPA-Y26
QSEPELKLESVVIVSRHGVRAPTKATQLMQDVTPDAWPTWPVKLGELTPRGGELIAYLGHYWRQRLVADELLPNQTCPQSGQVAIIADVDERTRKTGEAFAAGLAPDCAITVHTQADTSSPDPLFNPLKTGVCQLDNANVTDAILERAGGSIADFTGHYQTAFRELERVLNFSQSNLCLKREKQDESCSLTQALPSELKVSADNVSLTGAVSLASMLTEIFLLQQAQGMPEPGWGRITDSHQWNTLLSLHNAQFDLLQRTPEVARSRATPLLDLIKTALTPNGTQKQAYGVTLPTKVLFIAGHDTNLANLGGALELNWTLPGQPDNTPPGGELVFERWRRLSDNSCWIQVSLVFQTLQQMRDKTPLSLNTPPGEVKLTLAGCEERNAQGMCSCAGFTQIVNEARIPACSL

SEQ ID NO: 29 - protein, 410 aa, Artificial Sequence
  APPA-Y27
QSEPELKLESVVIVSRHGVRAPTKATQLMQDVTPDAWPTWPVKLGELTPRGGELIAYLGHYWRQRLVADELLPNQTCPQSGQVAIIADVDERTRKTGEAFAAGLAPDCAITVHTQADTSSPDPLFNPLKTGVCQLDNANVTDAILERAGGSIADFTGHYQTAFRELERVLNFSQSNLCLKREKQDESCSLTQALPSELKVSADNVSLTGAVSLASMLTEIFLLQQAQGMPEPGWGRITDSHQWNTLLSLHNAQFDLLQRTPEVARSRATPLLDLIKTALTPNGTQKQAYGVTLPTSVLFLAGHDTNLANLGGALELNWTLPGQPDNTPPGGELVFERWRRLSDNSCWIQVSLVFQTLQQMRDKTPLSLNTPPGEVKLTLAGCEERNAQGMCSCAGFTQIVNEARIPACSL

SEQ ID NO: 30 - protein, 410 aa, Artificial Sequence
  APPA-Y28
QSEPELKLESVVIVSRHGVRAPTKATQLMQDVTPDAWPTWPVKLGELTPRGGELIAYLGHYWRQRLVADELLPNQTCPQSGQVAIIADVDERTRKTGEAFAAGLAPDCAITVHTQADTSSPDPLFNPLKTGVCQLDNANVTDAILERAGGSIADFTGHYQTAFRELERVLNFSQSNLCLKREKQDESCSLTQALPSELKVSADNVSLTGAVSLASMLTEIFLLQQAQGMPEPGWGRITDSHQWNTLLSLHNAQFDLLQRTPEVARSRATPLLDLIKTALTPNGTQKQAYGVTLPTSVLFIAGHDTNIANLGGALELNWTLPGQPDNTPPGGELVFERWRRLSDNSCWIQVSLVFQTLQQMRDKTPLSLNTPPGEVKLTLAGCEERNAQGMCSCAGFTQIVNEARIPACSL

SEQ ID NO: 31 - protein, 410 aa, Artificial Sequence
  APPA-Y29
QSEPELKLESVVIVSRHGVRAPTKATQLMQDVTPDAWPTWPVKLGELTPRGGELIAYLGHYWRQRLVADELLPNQTCPQSGQVAIIADVDERTRKTGEAFAAGLAPDCAITVHTQADTSSPDPLFNPLKTGVCQLDNANVTDAILERAGGSIADFTGHYQTAFRELERVLNFSQSNLCLKREKQDESCSLTQALPSELKVSADNVSLTGAVSLASMLTEIFLLQQAQGMPEPGWGRITDSHQWNTLLSLHNAQFDLLQRTPEVARSRATPLLDLIKTALTPNGTQKQAYGVTLPTSVLFIAGHDTNLANLGGALELNWTLPGQPDNTPPGGELVFERWRRLSDNSFWIQVSLVFQTLQQMRDKTPLSLNTPPGEVKLTLAGCEERNAQGMCSCAGFTQIVNEARIPACSL

SEQ ID NO: 32 - protein, 410 aa, Artificial Sequence
  APPA-Y30
QSEPELKLESVVIVSRHGVRAPTKATQLMQDVTPDAWPTWPVKLGELTPRGGELIAYLGHYWRQRLVADELLPNQTCPQSGQVAIIADVDERTRKTGEAFAAGLAPDCAITVHTQADTSSPDPLFNPLKTGVCQLDNANVTDAILERAGGSIADFTGHYQTAFRELERVLNFSQSNLCLKREKQDESCSLTQALPSELKVSADNVSLTGAVSLASMLTEIFLLQQAQGMPEPGWGRITDSHQWNTLLSLHNAQFDLLQRTPEVARSRATPLLDLIKTALTPNGTQKQAYGVTLPTSVLFIAGHDTNLANLGGALELNWTLPGQPDNTPPGGELVFERWRRLSDNSCWIKVSLVFQTLQQMRDKTPLSLNTPPGEVKLTLAGCEERNAQGMCSCAGFTQIVNEARIPACSL

SEQ ID NO: 33 - protein, 410 aa, Artificial Sequence
  APPA-Y31
QSEPELKLESVVIVSRHGVRAPTKATQLMQDVTPDAWPTWPVKLGELTPRGGELIAYLGHYWRQRLVADELLPNQTCPQSGQVAIIADVDERTRKTGEAFAAGLAPDCAITVHTQADTSSPDPLFNPLKTGVCQLDNANVTDAILERAGGSIADFTGHYQTAFRELERVLNFSQSNLCLKREKQDESCSLTQALPSELKVSADNVSLTGAVSLASMLTEIFLLQQAQGMPEPGWGRITDSHQWNTLLSLHNAQFDLLQRTPEVARSRATPLLDLIKTALTPNGTQKQAYGVTLPTSVLFIAGHDTNLANLGGALELNWTLPGQPDNTPPGGELVFERWRRLSDNSCWIQVSYVFQTLQQMRDKTPLSLNTPPGEVKLTLAGCEERNAQGMCSCAGFTQIVNEARIPACSL

SEQ ID NO: 34 - protein, 410 aa, Artificial Sequence
  APPA-Y32
QSEPELKLESVVIVSRHGVRAPTKATQLMQDVTPDAWPTWPVKLGELTPRGGELIAYLGHYWRQRLVADELLPNQTCPQSGQVAIIADVDERTRKTGEAFAAGLAPDCAITVHTQADTSSPDPLFNPLKTGVCQLDNANVTDAILERAGGSIADFTGHYQTAFRELERVLNFSQSNLCLKREKQDESCSLTQALPSELKVSADNVSLTGAVSLASMLTEIFLLQQAQGMPEPGWGRITDSHQWNTLLSLHNAQFDLLQRTPEVARSRATPLLDLIKTALTPNGTQKQAYGVTLPTSVLFIAGHDTNLANLGGALELNWTLPGQPDNTPPGGELVFERWRRLSDNSCWIQVSLVYQTLQQMRDKTPLSLNTPPGEVKLTLAGCEERNAQGMCSCAGFTQIVNEARIPACSL

SEQ ID NO: 35 - protein, 410 aa, Artificial Sequence
  APPA-Y33
QSEPELKLESVVIVSRHGVRAPTKATQLMQDVTPDAWPTWPVKLGELTPRGGELIAYLGHYWRQRLVADELLPNQTCPQSGQVAIIADVDERTRKTGEAFAAGLAPDCAITVHTQADTSSPDPLFNPLKTGVCQLDNANVTDAILERAGGSIADFTGHYQTAFRELERVLNFSQSNLCLKREKQDESCSLTQALPSELKVSADNVSLTGAVSLASMLTEIFLLQQAQGMPEPGWGRITDSHQWNTLLSLHNAQFDLLQRTPEVARSRATPLLDLIKTALTPNGTQKQAYGVTLPTSVLFIAGHDTNLANLGGALELNWTLPGQPDNTPPGGELVFERWRRLSDNSCWIQVSLVFQTLQQLRDKTPLSLNTPPGEVKLTLAGCEERNAQGMCSCAGFTQIVNEARIPACSL

SEQ ID NO: 36 - protein, 410 aa, Artificial Sequence
  APPA-Y34
QSEPELKLESVVIVSRHGVRAPTKATQLMQDVTPDAWPTWPVKLGELTPRGGELIAYLGHYWRQRLVADELLPNQTCPQSGQVAIIADVDERTRKTGEAFAAGLAPDCAITVHTQADTSSPDPLFNPLKTGVCQLDNANVTDAILERAGGSIADFTGHYQTAFRELERVLNFSQSNLCLKREKQDESCSLTQALPSELKVSADNVSLTGAVSLASMLTEIFLLQQAQGMPEPGWGRITDSHQWNTLLSLHNAQFDLLQRTPEVARSRATPLLDLIKTALTPNGTQKQAYGVTLPTSVLFIAGHDTNLANLGGALELNWTLPGQPDNTPPGGELVFERWRRLSDNSCWIQVSLVFQTLQQMRDATPLSLNTPPGEVKLTLAGCEERNAQGMCSCAGFTQIVNEARIPACSL

SEQ ID NO: 37 - protein, 410 aa, Artificial Sequence
  APPA-Y35
QSEPELKLESVVIVSRHGVRAPTKATQLMQDVTPDAWPTWPVKLGELTPRGGELIAYLGHYWRQRLVADELLPNQTCPQSGQVAIIADVDERTRKTGEAFAAGLAPDCAITVHTQADTSSPDPLFNPLKTGVCQLDNANVTDAILERAGGSIADFTGHYQTAFRELERVLNFSQSNLCLKREKQDESCSLTQALPSELKVSADNVSLTGAVSLASMLTEIFLLQQAQGMPEPGWGRITDSHQWNTLLSLHNAQFDLLQRTPEVARSRATPLLDLIKTALTPNGTQKQAYGVTLPTSVLFIAGHDTNLANLGGALELNWTLPGQPDNTPPGGELVFERWRRLSDNSCWIQVSLVFQTLQQMRDKTPLSLNCPPGEVKLTLAGCEERNAQGMCSCAGFTQIVNEARIPACSL

SEQ ID NO: 38 - protein, 410 aa, Artificial Sequence
  APPA-Y36
QSEPELKLESVVIVSRHGVRAPTKATQLMQDVTPDAWPTWPVKLGELTPRGGELIAYLGHYWRQRLVADELLPNQTCPQSGQVAIIADVDERTRKTGEAFAAGLAPDCAITVHTQADTSSPDPLFNPLKTGVCQLDNANVTDAILERAGGSIADFTGHYQTAFRELERVLNFSQSNLCLKREKQDESCSLTQALPSELKVSADNVSLTGAVSLASMLTEIFLLQQAQGMPEPGWGRITDSHQWNTLLSLHNAQFDLLQRTPEVARSRATPLLDLIKTALTPNGTQKQAYGVTLPTSVLFIAGHDTNLANLGGALELNWTLPGQPDNTPPGGELVFERWRRLSDNSCWIQVSLVFQTLQQMRDKTPLSLNTPPGRVKLTLAGCEERNAQGMCSCAGFTQIVNEARIPACSL

SEQ ID NO: 39 - protein, 410 aa, Artificial Sequence
  APPA-Y37
QSEPELKLESVVIVSRHGVRAPTKATQLMQDVTPDAWPTWPVKLGELTPRGGELIAYLGHYWRQRLVADELLPNQTCPQSGQVAIIADVDERTRKTGEAFAAGLAPDCAITVHTQADTSSPDPLFNPLKTGVCQLDNANVTDAILERAGGSIADFTGHYQTAFRELERVLNFSQSNLCLKREKQDESCSLTQALPSELKVSADNVSLTGAVSLASMLTEIFLLQQAQGMPEPGWGRITDSHQWNTLLSLHNAQFDLLQRTPEVARSRATPLLDLIKTALTPNGTQKQAYGVTLPTSVLFIAGHDTNLANLGGALELNWTLPGQPDNTPPGGELVFERWRRLSDNSCWIQVSLVFQTLQQMRDKTPLSLNTPPGEVKLTLAGCEERNAQGMCSCAGFIQIVNEARIPACSL

SEQ ID NO: 40 - protein, 410 aa, Artificial Sequence
  APPA-Y38
QSEPELKLESVVIVSRHGVRAPTKATQLMQDVTPDAWPTWPVKLGELTPRGGELIAYLGHYWRQRLVADELLPNQTCPQSGQVAIIADVDERTRKTGEAFAAGLAPDCAITVHTQADTSSPDPLFNPLKTGVCQLDNANVTDAILERAGGSIADFTGHYQTAFRELERVLNFSQSNLCLKREKQDESCSLTQALPSELKVSADNVSLTGAVSLASMLTEIFLLQQAQGMPEPGWGRITDSHQWNTLLSLHNAQFDLLQRTPEVARSRATPLLDLIKTALTPNGTQKQAYGVTLPPSVLFIAGHDTNLANLGGALELNWTLPGQPDNTPPGGELVFERWRRLSDNSCWIKVSLVFQTLQQMRDKTPLSLNTPPGEVKLTLAGCEERNAQGMCSCAGFTQIVNEARIPACSL

SEQ ID NO: 41 - protein, 410 aa, Artificial Sequence
  APPA-Y39
QSEPELKLESVVIVSRHGVRAPTKATQLMQDVTPDAWPTWPVKLGELTPRGGELIAYLGHYWRQRLVADELLPNQTCPQSGQVAIIADVDERTRKTGEAFAAGLAPDCAITVHTQADTSSPDPLFNPLKTGVCQLDNANVTDAILERAGGSIADFTGHYQTAFRELERVLNFSQSNLCLKREKQDESCSLTQALPSELKVSADNVSLTGAVSLASMLTEIFLLQQAQGMPEPGWGRITDSHQWNTLLSLHNAQFDLLQRTPEVARSRATPLLDLIKTALTPNGTQKQAYGVTLPPSVLFIAGHDTNLANLGGALELNWTLPGQPDNTPPGGELVFERWRRLSDNSCWIQVSLVFQTLQQMRDKTPLSLNTPPGRVKLTLAGCEERNAQGMCSCAGFTQIVNEARIPACSL

SEQ ID NO: 42 - protein, 410 aa, Artificial Sequence
  APPA-Y40
QSEPELKLESVVIVSRHGVRAPTKATQLMQDVTPDAWPTWPVKLGELTPRGGELIAYLGHYWRQRLVADELLPNQTCPQSGQVAIIADVDERTRKTGEAFAAGLAPDCAITVHTQADTSSPDPLFNPLKTGVCQLDNANVTDAILERAGGSIADFTGHYQTAFRELERVLNFSQSNLCLKREKQDESCSLTQALPSELKVSADNVSLTGAVSLASMLTEIFLLQQAQGMPEPGWGRITDSHQWNTLLSLHNAQFDLLQRTPEVARSRATPLLDLIKTALTPNGTQKQAYGVTLPTSVLFIAGHDTNLANLGGALELNWTLPGQPDNTPPGGELVFERWRRLSDNSCWIKVSLVFQTLQQMRDKTPLSLNTPPGRVKLTLAGCEERNAQGMCSCAGFTQIVNEARIPACSL

SEQ ID NO: 43 - protein, 410 aa, Artificial Sequence
  APPA-Y41
QSEPELKLESVVIVSRHGVRAPTKATQLMQDVTPDAWPTWPVKLGELTPRGGELIAYLGHYWRQRLVADELLPNQTCPQSGQVAIIADVDERTRKTGEAFAAGLAPDCAITVHTQADTSSPDPLFNPLKTGVCQLDNANVTDAILERAGGSIADFTGHYQTAFRELERVLNFSQSNLCLKREKQDESCSLTQALPSELKVSADNVSLTGAVSLASMLTEIFLLQQAQGMPEPGWGRITDSHQWNTLLSLHNAQFDLLQRTPEVARSRATPLLDLIKTALTPNGTQKQAYGVTLPPSVLFIAGHDTNLANLGGALELNWTLPGQPDNTPPGGELVFERWRRLSDNSCWIKVSLVFQTLQQMRDKTPLSLNTPPGRVKLTLAGCEERNAQGMCSCAGFTQIVNEARIPACSL

SEQ ID NO: 44 - protein, 410 aa, Artificial Sequence
  APPA-Y25-1
QSEPELKLESVVIVSRHGVRAPTKATQLMQDVTPDAWPTWPVKLGELTPRGGELIAYLGHYWRQRLVADELLPNQTCPQSGQVAIIADVDERTRKTGEAFAAGLAPDCAITVHTQADTSSPDPLFNPLKTGVCQLDNANVTDAILERAGGSIADFTGHYQTAFRELERVLNFSQSNLCLKREKQDESCSLTQALPSELKVSADNVSLTGAVSLASMLTEIFLLQQAQGMPEPGWGRITDSHQWNTLLSLHNAQFDLLQRTPEVARSRATPLLDLIKTALTPNGTQKQAYGVTLPASVLFIAGHDTNLANLGGALELNWTLPGQPDNTPPGGELVFERWRRLSDNSCWIQVSLVFQTLQQMRDKTPLSLNTPPGEVKLTLAGCEERNAQGMCSCAGFTQIVNEARIPACSL

SEQ ID NO: 45 - protein, 410 aa, Artificial Sequence
  APPA-Y25-2
QSEPELKLESVVIVSRHGVRAPTKATQLMQDVTPDAWPTWPVKLGELTPRGGELIAYLGHYWRQRLVADELLPNQTCPQSGQVAIIADVDERTRKTGEAFAAGLAPDCAITVHTQADTSSPDPLFNPLKTGVCQLDNANVTDAILERAGGSIADFTGHYQTAFRELERVLNFSQSNLCLKREKQDESCSLTQALPSELKVSADNVSLTGAVSLASMLTEIFLLQQAQGMPEPGWGRITDSHQWNTLLSLHNAQFDLLQRTPEVARSRATPLLDLIKTALTPNGTQKQAYGVTLPCSVLFIAGHDTNLANLGGALELNWTLPGQPDNTPPGGELVFERWRRLSDNSCWIQVSLVFQTLQQMRDKTPLSLNTPPGEVKLTLAGCEERNAQGMCSCAGFTQIVNEARIPACSL

SEQ ID NO: 46 - protein, 410 aa, Artificial Sequence
  APPA-Y25-3
QSEPELKLESVVIVSRHGVRAPTKATQLMQDVTPDAWPTWPVKLGELTPRGGELIAYLGHYWRQRLVADELLPNQTCPQSGQVAIIADVDERTRKTGEAFAAGLAPDCAITVHTQADTSSPDPLFNPLKTGVCQLDNANVTDAILERAGGSIADFTGHYQTAFRELERVLNFSQSNLCLKREKQDESCSLTQALPSELKVSADNVSLTGAVSLASMLTEIFLLQQAQGMPEPGWGRITDSHQWNTLLSLHNAQFDLLQRTPEVARSRATPLLDLIKTALTPNGTQKQAYGVTLPDSVLFIAGHDTNLANLGGALELNWTLPGQPDNTPPGGELVFERWRRLSDNSCWIQVSLVFQTLQQMRDKTPLSLNTPPGEVKLTLAGCEERNAQGMCSCAGFTQIVNEARIPACSL

SEQ ID NO: 47 - protein, 410 aa, Artificial Sequence
  APPA-Y25-4
QSEPELKLESVVIVSRHGVRAPTKATQLMQDVTPDAWPTWPVKLGELTPRGGELIAYLGHYWRQRLVADELLPNQTCPQSGQVAIIADVDERTRKTGEAFAAGLAPDCAITVHTQADTSSPDPLFNPLKTGVCQLDNANVTDAILERAGGSIADFTGHYQTAFRELERVLNFSQSNLCLKREKQDESCSLTQALPSELKVSADNVSLTGAVSLASMLTEIFLLQQAQGMPEPGWGRITDSHQWNTLLSLHNAQFDLLQRTPEVARSRATPLLDLIKTALTPNGTQKQAYGVTLPESVLFIAGHDTNLANLGGALELNWTLPGQPDNTPPGGELVFERWRRLSDNSCWIQVSLVFQTLQQMRDKTPLSLNTPPGEVKLTLAGCEERNAQGMCSCAGFTQIVNEARIPACSL

SEQ ID NO: 48 - protein, 410 aa, Artificial Sequence
  APPA-Y25-5
QSEPELKLESVVIVSRHGVRAPTKATQLMQDVTPDAWPTWPVKLGELTPRGGELIAYLGHYWRQRLVADELLPNQTCPQSGQVAIIADVDERTRKTGEAFAAGLAPDCAITVHTQADTSSPDPLFNPLKTGVCQLDNANVTDAILERAGGSIADFTGHYQTAFRELERVLNFSQSNLCLKREKQDESCSLTQALPSELKVSADNVSLTGAVSLASMLTEIFLLQQAQGMPEPGWGRITDSHQWNTLLSLHNAQFDLLQRTPEVARSRATPLLDLIKTALTPNGTQKQAYGVTLPFSVLFIAGHDTNLANLGGALELNWTLPGQPDNTPPGGELVFERWRRLSDNSCWIQVSLVFQTLQQMRDKTPLSLNTPPGEVKLTLAGCEERNAQGMCSCAGFTQIVNEARIPACSL

SEQ ID NO: 49 - protein, 410 aa, Artificial Sequence
  APPA-Y25-6
QSEPELKLESVVIVSRHGVRAPTKATQLMQDVTPDAWPTWPVKLGELTPRGGELIAYLGHYWRQRLVADELLPNQTCPQSGQVAIIADVDERTRKTGEAFAAGLAPDCAITVHTQADTSSPDPLFNPLKTGVCQLDNANVTDAILERAGGSIADFTGHYQTAFRELERVLNFSQSNLCLKREKQDESCSLTQALPSELKVSADNVSLTGAVSLASMLTEIFLLQQAQGMPEPGWGRITDSHQWNTLLSLHNAQFDLLQRTPEVARSRATPLLDLIKTALTPNGTQKQAYGVTLPGSVLFIAGHDTNLANLGGALELNWTLPGQPDNTPPGGELVFERWRRLSDNSCWIQVSLVFQTLQQMRDKTPLSLNTPPGEVKLTLAGCEERNAQGMCSCAGFTQIVNEARIPACSL

SEQ ID NO: 50 - protein, 410 aa, Artificial Sequence
  APPA-Y25-7
QSEPELKLESVVIVSRHGVRAPTKATQLMQDVTPDAWPTWPVKLGELTPRGGELIAYLGHYWRQRLVADELLPNQTCPQSGQVAIIADVDERTRKTGEAFAAGLAPDCAITVHTQADTSSPDPLFNPLKTGVCQLDNANVTDAILERAGGSIADFTGHYQTAFRELERVLNFSQSNLCLKREKQDESCSLTQALPSELKVSADNVSLTGAVSLASMLTEIFLLQQAQGMPEPGWGRITDSHQWNTLLSLHNAQFDLLQRTPEVARSRATPLLDLIKTALTPNGTQKQAYGVTLPHSVLFIAGHDTNLANLGGALELNWTLPGQPDNTPPGGELVFERWRRLSDNSCWIQVSLVFQTLQQMRDKTPLSLNTPPGEVKLTLAGCEERNAQGMCSCAGFTQIVNEARIPACSL

SEQ ID NO: 51 - protein, 410 aa, Artificial Sequence
  APPA-Y25-8
QSEPELKLESVVIVSRHGVRAPTKATQLMQDVTPDAWPTWPVKLGELTPRGGELIAYLGHYWRQRLVADELLPNQTCPQSGQVAIIADVDERTRKTGEAFAAGLAPDCAITVHTQADTSSPDPLFNPLKTGVCQLDNANVTDAILERAGGSIADFTGHYQTAFRELERVLNFSQSNLCLKREKQDESCSLTQALPSELKVSADNVSLTGAVSLASMLTEIFLLQQAQGMPEPGWGRITDSHQWNTLLSLHNAQFDLLQRTPEVARSRATPLLDLIKTALTPNGTQKQAYGVTLPISVLFIAGHDTNLANLGGALELNWTLPGQPDNTPPGGELVFERWRRLSDNSCWIQVSLVFQTLQQMRDKTPLSLNTPPGEVKLTLAGCEERNAQGMCSCAGFTQIVNEARIPACSL

SEQ ID NO: 52 - protein, 410 aa, Artificial Sequence
  APPA-Y25-9
QSEPELKLESVVIVSRHGVRAPTKATQLMQDVTPDAWPTWPVKLGELTPRGGELIAYLGHYWRQRLVADELLPNQTCPQSGQVAIIADVDERTRKTGEAFAAGLAPDCAITVHTQADTSSPDPLFNPLKTGVCQLDNANVTDAILERAGGSIADFTGHYQTAFRELERVLNFSQSNLCLKREKQDESCSLTQALPSELKVSADNVSLTGAVSLASMLTEIFLLQQAQGMPEPGWGRITDSHQWNTLLSLHNAQFDLLQRTPEVARSRATPLLDLIKTALTPNGTQKQAYGVTLPKSVLFIAGHDTNLANLGGALELNWTLPGQPDNTPPGGELVFERWRRLSDNSCWIQVSLVFQTLQQMRDKTPLSLNTPPGEVKLTLAGCEERNAQGMCSCAGFTQIVNEARIPACSL

SEQ ID NO: 53 - protein, 410 aa, Artificial Sequence
  APPA-Y25-10
QSEPELKLESVVIVSRHGVRAPTKATQLMQDVTPDAWPTWPVKLGELTPRGGELIAYLGHYWRQRLVADELLPNQTCPQSGQVAIIADVDERTRKTGEAFAAGLAPDCAITVHTQADTSSPDPLFNPLKTGVCQLDNANVTDAILERAGGSIADFTGHYQTAFRELERVLNFSQSNLCLKREKQDESCSLTQALPSELKVSADNVSLTGAVSLASMLTEIFLLQQAQGMPEPGWGRITDSHQWNTLLSLHNAQFDLLQRTPEVARSRATPLLDLIKTALTPNGTQKQAYGVTLPLSVLFIAGHDTNLANLGGALELNWTLPGQPDNTPPGGELVFERWRRLSDNSCWIQVSLVFQTLQQMRDKTPLSLNTPPGEVKLTLAGCEERNAQGMCSCAGFTQIVNEARIPACSL

SEQ ID NO: 54 - protein, 410 aa, Artificial Sequence
  APPA-Y25-11
QSEPELKLESVVIVSRHGVRAPTKATQLMQDVTPDAWPTWPVKLGELTPRGGELIAYLGHYWRQRLVADELLPNQTCPQSGQVAIIADVDERTRKTGEAFAAGLAPDCAITVHTQADTSSPDPLFNPLKTGVCQLDNANVTDAILERAGGSIADFTGHYQTAFRELERVLNFSQSNLCLKREKQDESCSLTQALPSELKVSADNVSLTGAVSLASMLTEIFLLQQAQGMPEPGWGRITDSHQWNTLLSLHNAQFDLLQRTPEVARSRATPLLDLIKTALTPNGTQKQAYGVTLPMSVLFIAGHDTNLANLGGALELNWTLPGQPDNTPPGGELVFERWRRLSDNSCWIQVSLVFQTLQQMRDKTPLSLNTPPGEVKLTLAGCEERNAQGMCSCAGFTQIVNEARIPACSL

SEQ ID NO: 55 - protein, 410 aa, Artificial Sequence
  APPA-Y25-12
QSEPELKLESVVIVSRHGVRAPTKATQLMQDVTPDAWPTWPVKLGELTPRGGELIAYLGHYWRQRLVADELLPNQTCPQSGQVAIIADVDERTRKTGEAFAAGLAPDCAITVHTQADTSSPDPLFNPLKTGVCQLDNANVTDAILERAGGSIADFTGHYQTAFRELERVLNFSQSNLCLKREKQDESCSLTQALPSELKVSADNVSLTGAVSLASMLTEIFLLQQAQGMPEPGWGRITDSHQWNTLLSLHNAQFDLLQRTPEVARSRATPLLDLIKTALTPNGTQKQAYGVTLPNSVLFIAGHDTNLANLGGALELNWTLPGQPDNTPPGGELVFERWRRLSDNSCWIQVSLVFQTLQQMRDKTPLSLNTPPGEVKLTLAGCEERNAQGMCSCAGFTQIVNEARIPACSL

SEQ ID NO: 56 - protein, 410 aa, Artificial Sequence
  APPA-Y25-13
QSEPELKLESVVIVSRHGVRAPTKATQLMQDVTPDAWPTWPVKLGELTPRGGELIAYLGHYWRQRLVADELLPNQTCPQSGQVAIIADVDERTRKTGEAFAAGLAPDCAITVHTQADTSSPDPLFNPLKTGVCQLDNANVTDAILERAGGSIADFTGHYQTAFRELERVLNFSQSNLCLKREKQDESCSLTQALPSELKVSADNVSLTGAVSLASMLTEIFLLQQAQGMPEPGWGRITDSHQWNTLLSLHNAQFDLLQRTPEVARSRATPLLDLIKTALTPNGTQKQAYGVTLPQSVLFIAGHDTNLANLGGALELNWTLPGQPDNTPPGGELVFERWRRLSDNSCWIQVSLVFQTLQQMRDKTPLSLNTPPGEVKLTLAGCEERNAQGMCSCAGFTQIVNEARIPACSL

SEQ ID NO: 57 - protein, 410 aa, Artificial Sequence
  APPA-Y25-14
QSEPELKLESVVIVSRHGVRAPTKATQLMQDVTPDAWPTWPVKLGELTPRGGELIAYLGHYWRQRLVADELLPNQTCPQSGQVAIIADVDERTRKTGEAFAAGLAPDCAITVHTQADTSSPDPLFNPLKTGVCQLDNANVTDAILERAGGSIADFTGHYQTAFRELERVLNFSQSNLCLKREKQDESCSLTQALPSELKVSADNVSLTGAVSLASMLTEIFLLQQAQGMPEPGWGRITDSHQWNTLLSLHNAQFDLLQRTPEVARSRATPLLDLIKTALTPNGTQKQAYGVTLPRSVLFIAGHDTNLANLGGALELNWTLPGQPDNTPPGGELVFERWRRLSDNSCWIQVSLVFQTLQQMRDKTPLSLNTPPGEVKLTLAGCEERNAQGMCSCAGFTQIVNEARIPACSL

SEQ ID NO: 58 - protein, 410 aa, Artificial Sequence
  APPA-Y25-15
QSEPELKLESVVIVSRHGVRAPTKATQLMQDVTPDAWPTWPVKLGELTPRGGELIAYLGHYWRQRLVADELLPNQTCPQSGQVAIIADVDERTRKTGEAFAAGLAPDCAITVHTQADTSSPDPLFNPLKTGVCQLDNANVTDAILERAGGSIADFTGHYQTAFRELERVLNFSQSNLCLKREKQDESCSLTQALPSELKVSADNVSLTGAVSLASMLTEIFLLQQAQGMPEPGWGRITDSHQWNTLLSLHNAQFDLLQRTPEVARSRATPLLDLIKTALTPNGTQKQAYGVTLPSSVLFIAGHDTNLANLGGALELNWTLPGQPDNTPPGGELVFERWRRLSDNSCWIQVSLVFQTLQQMRDKTPLSLNTPPGEVKLTLAGCEERNAQGMCSCAGFTQIVNEARIPACSL

SEQ ID NO: 59 - protein, 410 aa, Artificial Sequence
  APPA-Y25-16
QSEPELKLESVVIVSRHGVRAPTKATQLMQDVTPDAWPTWPVKLGELTPRGGELIAYLGHYWRQRLVADELLPNQTCPQSGQVAIIADVDERTRKTGEAFAAGLAPDCAITVHTQADTSSPDPLFNPLKTGVCQLDNANVTDAILERAGGSIADFTGHYQTAFRELERVLNFSQSNLCLKREKQDESCSLTQALPSELKVSADNVSLTGAVSLASMLTEIFLLQQAQGMPEPGWGRITDSHQWNTLLSLHNAQFDLLQRTPEVARSRATPLLDLIKTALTPNGTQKQAYGVTLPVSVLFIAGHDTNLANLGGALELNWTLPGQPDNTPPGGELVFERWRRLSDNSCWIQVSLVFQTLQQMRDKTPLSLNTPPGEVKLTLAGCEERNAQGMCSCAGFTQIVNEARIPACSL

SEQ ID NO: 60 - protein, 410 aa, Artificial Sequence
  APPA-Y25-17
QSEPELKLESVVIVSRHGVRAPTKATQLMQDVTPDAWPTWPVKLGELTPRGGELIAYLGHYWRQRLVADELLPNQTCPQSGQVAIIADVDERTRKTGEAFAAGLAPDCAITVHTQADTSSPDPLFNPLKTGVCQLDNANVTDAILERAGGSIADFTGHYQTAFRELERVLNFSQSNLCLKREKQDESCSLTQALPSELKVSADNVSLTGAVSLASMLTEIFLLQQAQGMPEPGWGRITDSHQWNTLLSLHNAQFDLLQRTPEVARSRATPLLDLIKTALTPNGTQKQAYGVTLPWSVLFIAGHDTNLANLGGALELNWTLPGQPDNTPPGGELVFERWRRLSDNSCWIQVSLVFQTLQQMRDKTPLSLNTPPGEVKLTLAGCEERNAQGMCSCAGFTQIVNEARIPACSL

SEQ ID NO: 61 - protein, 410 aa, Artificial Sequence
  APPA-Y25-18
QSEPELKLESVVIVSRHGVRAPTKATQLMQDVTPDAWPTWPVKLGELTPRGGELIAYLGHYWRQRLVADELLPNQTCPQSGQVAIIADVDERTRKTGEAFAAGLAPDCAITVHTQADTSSPDPLFNPLKTGVCQLDNANVTDAILERAGGSIADFTGHYQTAFRELERVLNFSQSNLCLKREKQDESCSLTQALPSELKVSADNVSLTGAVSLASMLTEIFLLQQAQGMPEPGWGRITDSHQWNTLLSLHNAQFDLLQRTPEVARSRATPLLDLIKTALTPNGTQKQAYGVTLPYSVLFIAGHDTNLANLGGALELNWTLPGQPDNTPPGGELVFERWRRLSDNSCWIQVSLVFQTLQQMRDKTPLSLNTPPGEVKLTLAGCEERNAQGMCSCAGFTQIVNEARIPACSL

SEQ ID NO: 62 - protein, 410 aa, Artificial Sequence
  APPA-Y30-1
QSEPELKLESVVIVSRHGVRAPTKATQLMQDVTPDAWPTWPVKLGELTPRGGELIAYLGHYWRQRLVADELLPNQTCPQSGQVAIIADVDERTRKTGEAFAAGLAPDCAITVHTQADTSSPDPLFNPLKTGVCQLDNANVTDAILERAGGSIADFTGHYQTAFRELERVLNFSQSNLCLKREKQDESCSLTQALPSELKVSADNVSLTGAVSLASMLTEIFLLQQAQGMPEPGWGRITDSHQWNTLLSLHNAQFDLLQRTPEVARSRATPLLDLIKTALTPNGTQKQAYGVTLPTSVLFIAGHDTNLANLGGALELNWTLPGQPDNTPPGGELVFERWRRLSDNSCWIAVSLVFQTLQQMRDKTPLSLNTPPGEVKLTLAGCEERNAQGMCSCAGFTQIVNEARIPACSL

SEQ ID NO: 63 - protein, 410 aa, Artificial Sequence
  APPA-Y30-2
QSEPELKLESVVIVSRHGVRAPTKATQLMQDVTPDAWPTWPVKLGELTPRGGELIAYLGHYWRQRLVADELLPNQTCPQSGQVAIIADVDERTRKTGEAFAAGLAPDCAITVHTQADTSSPDPLFNPLKTGVCQLDNANVTDAILERAGGSIADFTGHYQTAFRELERVLNFSQSNLCLKREKQDESCSLTQALPSELKVSADNVSLTGAVSLASMLTEIFLLQQAQGMPEPGWGRITDSHQWNTLLSLHNAQFDLLQRTPEVARSRATPLLDLIKTALTPNGTQKQAYGVTLPTSVLFIAGHDTNLANLGGALELNWTLPGQPDNTPPGGELVFERWRRLSDNSCWICVSLVFQTLQQMRDKTPLSLNTPPGEVKLTLAGCEERNAQGMCSCAGFTQIVNEARIPACSL

SEQ ID NO: 64 - protein, 410 aa, Artificial Sequence
  APPA-Y30-3
QSEPELKLESVVIVSRHGVRAPTKATQLMQDVTPDAWPTWPVKLGELTPRGGELIAYLGHYWRQRLVADELLPNQTCPQSGQVAIIADVDERTRKTGEAFAAGLAPDCAITVHTQADTSSPDPLFNPLKTGVCQLDNANVTDAILERAGGSIADFTGHYQTAFRELERVLNFSQSNLCLKREKQDESCSLTQALPSELKVSADNVSLTGAVSLASMLTEIFLLQQAQGMPEPGWGRITDSHQWNTLLSLHNAQFDLLQRTPEVARSRATPLLDLIKTALTPNGTQKQAYGVTLPTSVLFIAGHDTNLANLGGALELNWTLPGQPDNTPPGGELVFERWRRLSDNSCWIDVSLVFQTLQQMRDKTPLSLNTPPGEVKLTLAGCEERNAQGMCSCAGFTQIVNEARIPACSL

SEQ ID NO: 65 - protein, 410 aa, Artificial Sequence
  APPA-Y30-4
QSEPELKLESVVIVSRHGVRAPTKATQLMQDVTPDAWPTWPVKLGELTPRGGELIAYLGHYWRQRLVADELLPNQTCPQSGQVAIIADVDERTRKTGEAFAAGLAPDCAITVHTQADTSSPDPLFNPLKTGVCQLDNANVTDAILERAGGSIADFTGHYQTAFRELERVLNFSQSNLCLKREKQDESCSLTQALPSELKVSADNVSLTGAVSLASMLTEIFLLQQAQGMPEPGWGRITDSHQWNTLLSLHNAQFDLLQRTPEVARSRATPLLDLIKTALTPNGTQKQAYGVTLPTSVLFIAGHDTNLANLGGALELNWTLPGQPDNTPPGGELVFERWRRLSDNSCWIEVSLVFQTLQQMRDKTPLSLNTPPGEVKLTLAGCEERNAQGMCSCAGFTQIVNEARIPACSL

SEQ ID NO: 66 - protein, 410 aa, Artificial Sequence
  APPA-Y30-5
QSEPELKLESVVIVSRHGVRAPTKATQLMQDVTPDAWPTWPVKLGELTPRGGELIAYLGHYWRQRLVADELLPNQTCPQSGQVAIIADVDERTRKTGEAFAAGLAPDCAITVHTQADTSSPDPLFNPLKTGVCQLDNANVTDAILERAGGSIADFTGHYQTAFRELERVLNFSQSNLCLKREKQDESCSLTQALPSELKVSADNVSLTGAVSLASMLTEIFLLQQAQGMPEPGWGRITDSHQWNTLLSLHNAQFDLLQRTPEVARSRATPLLDLIKTALTPNGTQKQAYGVTLPTSVLFIAGHDTNLANLGGALELNWTLPGQPDNTPPGGELVFERWRRLSDNSCWIFVSLVFQTLQQMRDKTPLSLNTPPGEVKLTLAGCEERNAQGMCSCAGFTQIVNEARIPACSL

SEQ ID NO: 67 - protein, 410 aa, Artificial Sequence
  APPA-Y30-6
QSEPELKLESVVIVSRHGVRAPTKATQLMQDVTPDAWPTWPVKLGELTPRGGELIAYLGHYWRQRLVADELLPNQTCPQSGQVAIIADVDERTRKTGEAFAAGLAPDCAITVHTQADTSSPDPLFNPLKTGVCQLDNANVTDAILERAGGSIADFTGHYQTAFRELERVLNFSQSNLCLKREKQDESCSLTQALPSELKVSADNVSLTGAVSLASMLTEIFLLQQAQGMPEPGWGRITDSHQWNTLLSLHNAQFDLLQRTPEVARSRATPLLDLIKTALTPNGTQKQAYGVTLPTSVLFIAGHDTNLANLGGALELNWTLPGQPDNTPPGGELVFERWRRLSDNSCWIGVSLVFQTLQQMRDKTPLSLNTPPGEVKLTLAGCEERNAQGMCSCAGFTQIVNEARIPACSL

SEQ ID NO: 68 - protein, 410 aa, Artificial Sequence
  APPA-Y30-7
QSEPELKLESVVIVSRHGVRAPTKATQLMQDVTPDAWPTWPVKLGELTPRGGELIAYLGHYWRQRLVADELLPNQTCPQSGQVAIIADVDERTRKTGEAFAAGLAPDCAITVHTQADTSSPDPLFNPLKTGVCQLDNANVTDAILERAGGSIADFTGHYQTAFRELERVLNFSQSNLCLKREKQDESCSLTQALPSELKVSADNVSLTGAVSLASMLTEIFLLQQAQGMPEPGWGRITDSHQWNTLLSLHNAQFDLLQRTPEVARSRATPLLDLIKTALTPNGTQKQAYGVTLPTSVLFIAGHDTNLANLGGALELNWTLPGQPDNTPPGGELVFERWRRLSDNSCWIHVSLVFQTLQQMRDKTPLSLNTPPGEVKLTLAGCEERNAQGMCSCAGFTQIVNEARIPACSL

SEQ ID NO: 69 - protein, 410 aa, Artificial Sequence
  APPA-Y30-8
QSEPELKLESVVIVSRHGVRAPTKATQLMQDVTPDAWPTWPVKLGELTPRGGELIAYLGHYWRQRLVADELLPNQTCPQSGQVAIIADVDERTRKTGEAFAAGLAPDCAITVHTQADTSSPDPLFNPLKTGVCQLDNANVTDAILERAGGSIADFTGHYQTAFRELERVLNFSQSNLCLKREKQDESCSLTQALPSELKVSADNVSLTGAVSLASMLTEIFLLQQAQGMPEPGWGRITDSHQWNTLLSLHNAQFDLLQRTPEVARSRATPLLDLIKTALTPNGTQKQAYGVTLPTSVLFIAGHDTNLANLGGALELNWTLPGQPDNTPPGGELVFERWRRLSDNSCWIIVSLVFQTLQQMRDKTPLSLNTPPGEVKLTLAGCEERNAQGMCSCAGFTQIVNEARIPACSL

SEQ ID NO: 70 - protein, 410 aa, Artificial Sequence
  APPA-Y30-9
QSEPELKLESVVIVSRHGVRAPTKATQLMQDVTPDAWPTWPVKLGELTPRGGELIAYLGHYWRQRLVADELLPNQTCPQSGQVAIIADVDERTRKTGEAFAAGLAPDCAITVHTQADTSSPDPLFNPLKTGVCQLDNANVTDAILERAGGSIADFTGHYQTAFRELERVLNFSQSNLCLKREKQDESCSLTQALPSELKVSADNVSLTGAVSLASMLTEIFLLQQAQGMPEPGWGRITDSHQWNTLLSLHNAQFDLLQRTPEVARSRATPLLDLIKTALTPNGTQKQAYGVTLPTSVLFIAGHDTNLANLGGALELNWTLPGQPDNTPPGGELVFERWRRLSDNSCWILVSLVFQTLQQMRDKTPLSLNTPPGEVKLTLAGCEERNAQGMCSCAGFTQIVNEARIPACSL

SEQ ID NO: 71 - protein, 410 aa, Artificial Sequence
  APPA-Y30-10
QSEPELKLESVVIVSRHGVRAPTKATQLMQDVTPDAWPTWPVKLGELTPRGGELIAYLGHYWRQRLVADELLPNQTCPQSGQVAIIADVDERTRKTGEAFAAGLAPDCAITVHTQADTSSPDPLFNPLKTGVCQLDNANVTDAILERAGGSIADFTGHYQTAFRELERVLNFSQSNLCLKREKQDESCSLTQALPSELKVSADNVSLTGAVSLASMLTEIFLLQQAQGMPEPGWGRITDSHQWNTLLSLHNAQFDLLQRTPEVARSRATPLLDLIKTALTPNGTQKQAYGVTLPTSVLFIAGHDTNLANLGGALELNWTLPGQPDNTPPGGELVFERWRRLSDNSCWIMVSLVFQTLQQMRDKTPLSLNTPPGEVKLTLAGCEERNAQGMCSCAGFTQIVNEARIPACSL

SEQ ID NO: 72 - protein, 410 aa, Artificial Sequence
  APPA-Y30-11
QSEPELKLESVVIVSRHGVRAPTKATQLMQDVTPDAWPTWPVKLGELTPRGGELIAYLGHYWRQRLVADELLPNQTCPQSGQVAIIADVDERTRKTGEAFAAGLAPDCAITVHTQADTSSPDPLFNPLKTGVCQLDNANVTDAILERAGGSIADFTGHYQTAFRELERVLNFSQSNLCLKREKQDESCSLTQALPSELKVSADNVSLTGAVSLASMLTEIFLLQQAQGMPEPGWGRITDSHQWNTLLSLHNAQFDLLQRTPEVARSRATPLLDLIKTALTPNGTQKQAYGVTLPTSVLFIAGHDTNLANLGGALELNWTLPGQPDNTPPGGELVFERWRRLSDNSCWINVSLVFQTLQQMRDKTPLSLNTPPGEVKLTLAGCEERNAQGMCSCAGFTQIVNEARIPACSL

SEQ ID NO: 73 - protein, 410 aa, Artificial Sequence
  APPA-Y30-12
QSEPELKLESVVIVSRHGVRAPTKATQLMQDVTPDAWPTWPVKLGELTPRGGELIAYLGHYWRQRLVADELLPNQTCPQSGQVAIIADVDERTRKTGEAFAAGLAPDCAITVHTQADTSSPDPLFNPLKTGVCQLDNANVTDAILERAGGSIADFTGHYQTAFRELERVLNFSQSNLCLKREKQDESCSLTQALPSELKVSADNVSLTGAVSLASMLTEIFLLQQAQGMPEPGWGRITDSHQWNTLLSLHNAQFDLLQRTPEVARSRATPLLDLIKTALTPNGTQKQAYGVTLPTSVLFIAGHDTNLANLGGALELNWTLPGQPDNTPPGGELVFERWRRLSDNSCWIPVSLVFQTLQQMRDKTPLSLNTPPGEVKLTLAGCEERNAQGMCSCAGFTQIVNEARIPACSL

SEQ ID NO: 74 - protein, 410 aa, Artificial Sequence
  APPA-Y30-13
QSEPELKLESVVIVSRHGVRAPTKATQLMQDVTPDAWPTWPVKLGELTPRGGELIAYLGHYWRQRLVADELLPNQTCPQSGQVAIIADVDERTRKTGEAFAAGLAPDCAITVHTQADTSSPDPLFNPLKTGVCQLDNANVTDAILERAGGSIADFTGHYQTAFRELERVLNFSQSNLCLKREKQDESCSLTQALPSELKVSADNVSLTGAVSLASMLTEIFLLQQAQGMPEPGWGRITDSHQWNTLLSLHNAQFDLLQRTPEVARSRATPLLDLIKTALTPNGTQKQAYGVTLPTSVLFIAGHDTNLANLGGALELNWTLPGQPDNTPPGGELVFERWRRLSDNSCWIRVSLVFQTLQQMRDKTPLSLNTPPGEVKLTLAGCEERNAQGMCSCAGFTQIVNEARIPACSL

SEQ ID NO: 75 - protein, 410 aa, Artificial Sequence
  APPA-Y30-14
QSEPELKLESVVIVSRHGVRAPTKATQLMQDVTPDAWPTWPVKLGELTPRGGELIAYLGHYWRQRLVADELLPNQTCPQSGQVAIIADVDERTRKTGEAFAAGLAPDCAITVHTQADTSSPDPLFNPLKTGVCQLDNANVTDAILERAGGSIADFTGHYQTAFRELERVLNFSQSNLCLKREKQDESCSLTQALPSELKVSADNVSLTGAVSLASMLTEIFLLQQAQGMPEPGWGRITDSHQWNTLLSLHNAQFDLLQRTPEVARSRATPLLDLIKTALTPNGTQKQAYGVTLPTSVLFIAGHDTNLANLGGALELNWTLPGQPDNTPPGGELVFERWRRLSDNSCWISVSLVFQTLQQMRDKTPLSLNTPPGEVKLTLAGCEERNAQGMCSCAGFTQIVNEARIPACSL

SEQ ID NO: 76 - protein, 410 aa, Artificial Sequence
  APPA-Y30-15
QSEPELKLESVVIVSRHGVRAPTKATQLMQDVTPDAWPTWPVKLGELTPRGGELIAYLGHYWRQRLVADELLPNQTCPQSGQVAIIADVDERTRKTGEAFAAGLAPDCAITVHTQADTSSPDPLFNPLKTGVCQLDNANVTDAILERAGGSIADFTGHYQTAFRELERVLNFSQSNLCLKREKQDESCSLTQALPSELKVSADNVSLTGAVSLASMLTEIFLLQQAQGMPEPGWGRITDSHQWNTLLSLHNAQFDLLQRTPEVARSRATPLLDLIKTALTPNGTQKQAYGVTLPTSVLFIAGHDTNLANLGGALELNWTLPGQPDNTPPGGELVFERWRRLSDNSCWITVSLVFQTLQQMRDKTPLSLNTPPGEVKLTLAGCEERNAQGMCSCAGFTQIVNEARIPACSL

SEQ ID NO: 77 - protein, 410 aa, Artificial Sequence
  APPA-Y30-16
QSEPELKLESVVIVSRHGVRAPTKATQLMQDVTPDAWPTWPVKLGELTPRGGELIAYLGHYWRQRLVADELLPNQTCPQSGQVAIIADVDERTRKTGEAFAAGLAPDCAITVHTQADTSSPDPLFNPLKTGVCQLDNANVTDAILERAGGSIADFTGHYQTAFRELERVLNFSQSNLCLKREKQDESCSLTQALPSELKVSADNVSLTGAVSLASMLTEIFLLQQAQGMPEPGWGRITDSHQWNTLLSLHNAQFDLLQRTPEVARSRATPLLDLIKTALTPNGTQKQAYGVTLPTSVLFIAGHDTNLANLGGALELNWTLPGQPDNTPPGGELVFERWRRLSDNSCWIVVSLVFQTLQQMRDKTPLSLNTPPGEVKLTLAGCEERNAQGMCSCAGFTQIVNEARIPACSL

SEQ ID NO: 78 - protein, 410 aa, Artificial Sequence
  APPA-Y30-17
QSEPELKLESVVIVSRHGVRAPTKATQLMQDVTPDAWPTWPVKLGELTPRGGELIAYLGHYWRQRLVADELLPNQTCPQSGQVAIIADVDERTRKTGEAFAAGLAPDCAITVHTQADTSSPDPLFNPLKTGVCQLDNANVTDAILERAGGSIADFTGHYQTAFRELERVLNFSQSNLCLKREKQDESCSLTQALPSELKVSADNVSLTGAVSLASMLTEIFLLQQAQGMPEPGWGRITDSHQWNTLLSLHNAQFDLLQRTPEVARSRATPLLDLIKTALTPNGTQKQAYGVTLPTSVLFIAGHDTNLANLGGALELNWTLPGQPDNTPPGGELVFERWRRLSDNSCWIWVSLVFQTLQQMRDKTPLSLNTPPGEVKLTLAGCEERNAQGMCSCAGFTQIVNEARIPACSL

SEQ ID NO: 79 - protein, 410 aa, Artificial Sequence
  APPA-Y30-18
QSEPELKLESVVIVSRHGVRAPTKATQLMQDVTPDAWPTWPVKLGELTPRGGELIAYLGHYWRQRLVADELLPNQTCPQSGQVAIIADVDERTRKTGEAFAAGLAPDCAITVHTQADTSSPDPLFNPLKTGVCQLDNANVTDAILERAGGSIADFTGHYQTAFRELERVLNFSQSNLCLKREKQDESCSLTQALPSELKVSADNVSLTGAVSLASMLTEIFLLQQAQGMPEPGWGRITDSHQWNTLLSLHNAQFDLLQRTPEVARSRATPLLDLIKTALTPNGTQKQAYGVTLPTSVLFIAGHDTNLANLGGALELNWTLPGQPDNTPPGGELVFERWRRLSDNSCWIYVSLVFQTLQQMRDKTPLSLNTPPGEVKLTLAGCEERNAQGMCSCAGFTQIVNEARIPACSL

SEQ ID NO: 80 - protein, 410 aa, Artificial Sequence
  APPA-Y36-1
QSEPELKLESVVIVSRHGVRAPTKATQLMQDVTPDAWPTWPVKLGELTPRGGELIAYLGHYWRQRLVADELLPNQTCPQSGQVAIIADVDERTRKTGEAFAAGLAPDCAITVHTQADTSSPDPLFNPLKTGVCQLDNANVTDAILERAGGSIADFTGHYQTAFRELERVLNFSQSNLCLKREKQDESCSLTQALPSELKVSADNVSLTGAVSLASMLTEIFLLQQAQGMPEPGWGRITDSHQWNTLLSLHNAQFDLLQRTPEVARSRATPLLDLIKTALTPNGTQKQAYGVTLPTSVLFIAGHDTNLANLGGALELNWTLPGQPDNTPPGGELVFERWRRLSDNSCWIQVSLVFQTLQQMRDKTPLSLNTPPGAVKLTLAGCEERNAQGMCSCAGFTQIVNEARIPACSL

SEQ ID NO: 81 - protein, 410 aa, Artificial Sequence
  APPA-Y36-2
QSEPELKLESVVIVSRHGVRAPTKATQLMQDVTPDAWPTWPVKLGELTPRGGELIAYLGHYWRQRLVADELLPNQTCPQSGQVAIIADVDERTRKTGEAFAAGLAPDCAITVHTQADTSSPDPLFNPLKTGVCQLDNANVTDAILERAGGSIADFTGHYQTAFRELERVLNFSQSNLCLKREKQDESCSLTQALPSELKVSADNVSLTGAVSLASMLTEIFLLQQAQGMPEPGWGRITDSHQWNTLLSLHNAQFDLLQRTPEVARSRATPLLDLIKTALTPNGTQKQAYGVTLPTSVLFIAGHDTNLANLGGALELNWTLPGQPDNTPPGGELVFERWRRLSDNSCWIQVSLVFQTLQQMRDKTPLSLNTPPGCVKLTLAGCEERNAQGMCSCAGFTQIVNEARIPACSL

SEQ ID NO: 82 - protein, 410 aa, Artificial Sequence
  APPA-Y36-3
QSEPELKLESVVIVSRHGVRAPTKATQLMQDVTPDAWPTWPVKLGELTPRGGELIAYLGHYWRQRLVADELLPNQTCPQSGQVAIIADVDERTRKTGEAFAAGLAPDCAITVHTQADTSSPDPLFNPLKTGVCQLDNANVTDAILERAGGSIADFTGHYQTAFRELERVLNFSQSNLCLKREKQDESCSLTQALPSELKVSADNVSLTGAVSLASMLTEIFLLQQAQGMPEPGWGRITDSHQWNTLLSLHNAQFDLLQRTPEVARSRATPLLDLIKTALTPNGTQKQAYGVTLPTSVLFIAGHDTNLANLGGALELNWTLPGQPDNTPPGGELVFERWRRLSDNSCWIQVSLVFQTLQQMRDKTPLSLNTPPGDVKLTLAGCEERNAQGMCSCAGFTQIVNEARIPACSL

SEQ ID NO: 83 - protein, 410 aa, Artificial Sequence
  APPA-Y36-4
QSEPELKLESVVIVSRHGVRAPTKATQLMQDVTPDAWPTWPVKLGELTPRGGELIAYLGHYWRQRLVADELLPNQTCPQSGQVAIIADVDERTRKTGEAFAAGLAPDCAITVHTQADTSSPDPLFNPLKTGVCQLDNANVTDAILERAGGSIADFTGHYQTAFRELERVLNFSQSNLCLKREKQDESCSLTQALPSELKVSADNVSLTGAVSLASMLTEIFLLQQAQGMPEPGWGRITDSHQWNTLLSLHNAQFDLLQRTPEVARSRATPLLDLIKTALTPNGTQKQAYGVTLPTSVLFIAGHDTNLANLGGALELNWTLPGQPDNTPPGGELVFERWRRLSDNSCWIQVSLVFQTLQQMRDKTPLSLNTPPGFVKLTLAGCEERNAQGMCSCAGFTQIVNEARIPACSL

SEQ ID NO: 84 - protein, 410 aa, Artificial Sequence
  APPA-Y36-5
QSEPELKLESVVIVSRHGVRAPTKATQLMQDVTPDAWPTWPVKLGELTPRGGELIAYLGHYWRQRLVADELLPNQTCPQSGQVAIIADVDERTRKTGEAFAAGLAPDCAITVHTQADTSSPDPLFNPLKTGVCQLDNANVTDAILERAGGSIADFTGHYQTAFRELERVLNFSQSNLCLKREKQDESCSLTQALPSELKVSADNVSLTGAVSLASMLTEIFLLQQAQGMPEPGWGRITDSHQWNTLLSLHNAQFDLLQRTPEVARSRATPLLDLIKTALTPNGTQKQAYGVTLPTSVLFIAGHDTNLANLGGALELNWTLPGQPDNTPPGGELVFERWRRLSDNSCWIQVSLVFQTLQQMRDKTPLSLNTPPGGVKLTLAGCEERNAQGMCSCAGFTQIVNEARIPACSL

SEQ ID NO: 85 - protein, 410 aa, Artificial Sequence
  APPA-Y36-6
QSEPELKLESVVIVSRHGVRAPTKATQLMQDVTPDAWPTWPVKLGELTPRGGELIAYLGHYWRQRLVADELLPNQTCPQSGQVAIIADVDERTRKTGEAFAAGLAPDCAITVHTQADTSSPDPLFNPLKTGVCQLDNANVTDAILERAGGSIADFTGHYQTAFRELERVLNFSQSNLCLKREKQDESCSLTQALPSELKVSADNVSLTGAVSLASMLTEIFLLQQAQGMPEPGWGRITDSHQWNTLLSLHNAQFDLLQRTPEVARSRATPLLDLIKTALTPNGTQKQAYGVTLPTSVLFIAGHDTNLANLGGALELNWTLPGQPDNTPPGGELVFERWRRLSDNSCWIQVSLVFQTLQQMRDKTPLSLNTPPGHVKLTLAGCEERNAQGMCSCAGFTQIVNEARIPACSL

SEQ ID NO: 86 - protein, 410 aa, Artificial Sequence
  APPA-Y36-7
QSEPELKLESVVIVSRHGVRAPTKATQLMQDVTPDAWPTWPVKLGELTPRGGELIAYLGHYWRQRLVADELLPNQTCPQSGQVAIIADVDERTRKTGEAFAAGLAPDCAITVHTQADTSSPDPLFNPLKTGVCQLDNANVTDAILERAGGSIADFTGHYQTAFRELERVLNFSQSNLCLKREKQDESCSLTQALPSELKVSADNVSLTGAVSLASMLTEIFLLQQAQGMPEPGWGRITDSHQWNTLLSLHNAQFDLLQRTPEVARSRATPLLDLIKTALTPNGTQKQAYGVTLPTSVLFIAGHDTNLANLGGALELNWTLPGQPDNTPPGGELVFERWRRLSDNSCWIQVSLVFQTLQQMRDKTPLSLNTPPGIVKLTLAGCEERNAQGMCSCAGFTQIVNEARIPACSL

SEQ ID NO: 87 - protein, 410 aa, Artificial Sequence
  APPA-Y36-8
QSEPELKLESVVIVSRHGVRAPTKATQLMQDVTPDAWPTWPVKLGELTPRGGELIAYLGHYWRQRLVADELLPNQTCPQSGQVAIIADVDERTRKTGEAFAAGLAPDCAITVHTQADTSSPDPLFNPLKTGVCQLDNANVTDAILERAGGSIADFTGHYQTAFRELERVLNFSQSNLCLKREKQDESCSLTQALPSELKVSADNVSLTGAVSLASMLTEIFLLQQAQGMPEPGWGRITDSHQWNTLLSLHNAQFDLLQRTPEVARSRATPLLDLIKTALTPNGTQKQAYGVTLPTSVLFIAGHDTNLANLGGALELNWTLPGQPDNTPPGGELVFERWRRLSDNSCWIQVSLVFQTLQQMRDKTPLSLNTPPGKVKLTLAGCEERNAQGMCSCAGFTQIVNEARIPACSL

SEQ ID NO: 88 - protein, 410 aa, Artificial Sequence
  APPA-Y36-9
QSEPELKLESVVIVSRHGVRAPTKATQLMQDVTPDAWPTWPVKLGELTPRGGELIAYLGHYWRQRLVADELLPNQTCPQSGQVAIIADVDERTRKTGEAFAAGLAPDCAITVHTQADTSSPDPLFNPLKTGVCQLDNANVTDAILERAGGSIADFTGHYQTAFRELERVLNFSQSNLCLKREKQDESCSLTQALPSELKVSADNVSLTGAVSLASMLTEIFLLQQAQGMPEPGWGRITDSHQWNTLLSLHNAQFDLLQRTPEVARSRATPLLDLIKTALTPNGTQKQAYGVTLPTSVLFIAGHDTNLANLGGALELNWTLPGQPDNTPPGGELVFERWRRLSDNSCWIQVSLVFQTLQQMRDKTPLSLNTPPGLVKLTLAGCEERNAQGMCSCAGFTQIVNEARIPACSL

SEQ ID NO: 89 - protein, 410 aa, Artificial Sequence
  APPA-Y36-10
QSEPELKLESVVIVSRHGVRAPTKATQLMQDVTPDAWPTWPVKLGELTPRGGELIAYLGHYWRQRLVADELLPNQTCPQSGQVAIIADVDERTRKTGEAFAAGLAPDCAITVHTQADTSSPDPLFNPLKTGVCQLDNANVTDAILERAGGSIADFTGHYQTAFRELERVLNFSQSNLCLKREKQDESCSLTQALPSELKVSADNVSLTGAVSLASMLTEIFLLQQAQGMPEPGWGRITDSHQWNTLLSLHNAQFDLLQRTPEVARSRATPLLDLIKTALTPNGTQKQAYGVTLPTSVLFIAGHDTNLANLGGALELNWTLPGQPDNTPPGGELVFERWRRLSDNSCWIQVSLVFQTLQQMRDKTPLSLNTPPGMVKLTLAGCEERNAQGMCSCAGFTQIVNEARIPACSL

SEQ ID NO: 90 - protein, 410 aa, Artificial Sequence
  APPA-Y36-11
QSEPELKLESVVIVSRHGVRAPTKATQLMQDVTPDAWPTWPVKLGELTPRGGELIAYLGHYWRQRLVADELLPNQTCPQSGQVAIIADVDERTRKTGEAFAAGLAPDCAITVHTQADTSSPDPLFNPLKTGVCQLDNANVTDAILERAGGSIADFTGHYQTAFRELERVLNFSQSNLCLKREKQDESCSLTQALPSELKVSADNVSLTGAVSLASMLTEIFLLQQAQGMPEPGWGRITDSHQWNTLLSLHNAQFDLLQRTPEVARSRATPLLDLIKTALTPNGTQKQAYGVTLPTSVLFIAGHDTNLANLGGALELNWTLPGQPDNTPPGGELVFERWRRLSDNSCWIQVSLVFQTLQQMRDKTPLSLNTPPGNVKLTLAGCEERNAQGMCSCAGFTQIVNEARIPACSL

SEQ ID NO: 91 - protein, 410 aa, Artificial Sequence
  APPA-Y36-12
QSEPELKLESVVIVSRHGVRAPTKATQLMQDVTPDAWPTWPVKLGELTPRGGELIAYLGHYWRQRLVADELLPNQTCPQSGQVAIIADVDERTRKTGEAFAAGLAPDCAITVHTQADTSSPDPLFNPLKTGVCQLDNANVTDAILERAGGSIADFTGHYQTAFRELERVLNFSQSNLCLKREKQDESCSLTQALPSELKVSADNVSLTGAVSLASMLTEIFLLQQAQGMPEPGWGRITDSHQWNTLLSLHNAQFDLLQRTPEVARSRATPLLDLIKTALTPNGTQKQAYGVTLPTSVLFIAGHDTNLANLGGALELNWTLPGQPDNTPPGGELVFERWRRLSDNSCWIQVSLVFQTLQQMRDKTPLSLNTPPGPVKLTLAGCEERNAQGMCSCAGFTQIVNEARIPACSL

SEQ ID NO: 92 - protein, 410 aa, Artificial Sequence
  APPA-Y36-13
QSEPELKLESVVIVSRHGVRAPTKATQLMQDVTPDAWPTWPVKLGELTPRGGELIAYLGHYWRQRLVADELLPNQTCPQSGQVAIIADVDERTRKTGEAFAAGLAPDCAITVHTQADTSSPDPLFNPLKTGVCQLDNANVTDAILERAGGSIADFTGHYQTAFRELERVLNFSQSNLCLKREKQDESCSLTQALPSELKVSADNVSLTGAVSLASMLTEIFLLQQAQGMPEPGWGRITDSHQWNTLLSLHNAQFDLLQRTPEVARSRATPLLDLIKTALTPNGTQKQAYGVTLPTSVLFIAGHDTNLANLGGALELNWTLPGQPDNTPPGGELVFERWRRLSDNSCWIQVSLVFQTLQQMRDKTPLSLNTPPGQVKLTLAGCEERNAQGMCSCAGFTQIVNEARIPACSL

SEQ ID NO: 93 - protein, 410 aa, Artificial Sequence
  APPA-Y36-14
QSEPELKLESVVIVSRHGVRAPTKATQLMQDVTPDAWPTWPVKLGELTPRGGELIAYLGHYWRQRLVADELLPNQTCPQSGQVAIIADVDERTRKTGEAFAAGLAPDCAITVHTQADTSSPDPLFNPLKTGVCQLDNANVTDAILERAGGSIADFTGHYQTAFRELERVLNFSQSNLCLKREKQDESCSLTQALPSELKVSADNVSLTGAVSLASMLTEIFLLQQAQGMPEPGWGRITDSHQWNTLLSLHNAQFDLLQRTPEVARSRATPLLDLIKTALTPNGTQKQAYGVTLPTSVLFIAGHDTNLANLGGALELNWTLPGQPDNTPPGGELVFERWRRLSDNSCWIQVSLVFQTLQQMRDKTPLSLNTPPGSVKLTLAGCEERNAQGMCSCAGFTQIVNEARIPACSL

SEQ ID NO: 94 - protein, 410 aa, Artificial Sequence
  APPA-Y36-15
QSEPELKLESVVIVSRHGVRAPTKATQLMQDVTPDAWPTWPVKLGELTPRGGELIAYLGHYWRQRLVADELLPNQTCPQSGQVAIIADVDERTRKTGEAFAAGLAPDCAITVHTQADTSSPDPLFNPLKTGVCQLDNANVTDAILERAGGSIADFTGHYQTAFRELERVLNFSQSNLCLKREKQDESCSLTQALPSELKVSADNVSLTGAVSLASMLTEIFLLQQAQGMPEPGWGRITDSHQWNTLLSLHNAQFDLLQRTPEVARSRATPLLDLIKTALTPNGTQKQAYGVTLPTSVLFIAGHDTNLANLGGALELNWTLPGQPDNTPPGGELVFERWRRLSDNSCWIQVSLVFQTLQQMRDKTPLSLNTPPGTVKLTLAGCEERNAQGMCSCAGFTQIVNEARIPACSL

SEQ ID NO: 95 - protein, 410 aa, Artificial Sequence
  APPA-Y36-16
QSEPELKLESVVIVSRHGVRAPTKATQLMQDVTPDAWPTWPVKLGELTPRGGELIAYLGHYWRQRLVADELLPNQTCPQSGQVAIIADVDERTRKTGEAFAAGLAPDCAITVHTQADTSSPDPLFNPLKTGVCQLDNANVTDAILERAGGSIADFTGHYQTAFRELERVLNFSQSNLCLKREKQDESCSLTQALPSELKVSADNVSLTGAVSLASMLTEIFLLQQAQGMPEPGWGRITDSHQWNTLLSLHNAQFDLLQRTPEVARSRATPLLDLIKTALTPNGTQKQAYGVTLPTSVLFIAGHDTNLANLGGALELNWTLPGQPDNTPPGGELVFERWRRLSDNSCWIQVSLVFQTLQQMRDKTPLSLNTPPGVVKLTLAGCEERNAQGMCSCAGFTQIVNEARIPACSL

SEQ ID NO: 96 - protein, 410 aa, Artificial Sequence
  APPA-Y36-17
QSEPELKLESVVIVSRHGVRAPTKATQLMQDVTPDAWPTWPVKLGELTPRGGELIAYLGHYWRQRLVADELLPNQTCPQSGQVAIIADVDERTRKTGEAFAAGLAPDCAITVHTQADTSSPDPLFNPLKTGVCQLDNANVTDAILERAGGSIADFTGHYQTAFRELERVLNFSQSNLCLKREKQDESCSLTQALPSELKVSADNVSLTGAVSLASMLTEIFLLQQAQGMPEPGWGRITDSHQWNTLLSLHNAQFDLLQRTPEVARSRATPLLDLIKTALTPNGTQKQAYGVTLPTSVLFIAGHDTNLANLGGALELNWTLPGQPDNTPPGGELVFERWRRLSDNSCWIQVSLVFQTLQQMRDKTPLSLNTPPGWVKLTLAGCEERNAQGMCSCAGFTQIVNEARIPACSL

SEQ ID NO: 97 - protein, 410 aa, Artificial Sequence
  APPA-Y36-18
QSEPELKLESVVIVSRHGVRAPTKATQLMQDVTPDAWPTWPVKLGELTPRGGELIAYLGHYWRQRLVADELLPNQTCPQSGQVAIIADVDERTRKTGEAFAAGLAPDCAITVHTQADTSSPDPLFNPLKTGVCQLDNANVTDAILERAGGSIADFTGHYQTAFRELERVLNFSQSNLCLKREKQDESCSLTQALPSELKVSADNVSLTGAVSLASMLTEIFLLQQAQGMPEPGWGRITDSHQWNTLLSLHNAQFDLLQRTPEVARSRATPLLDLIKTALTPNGTQKQAYGVTLPTSVLFIAGHDTNLANLGGALELNWTLPGQPDNTPPGGELVFERWRRLSDNSCWIQVSLVFQTLQQMRDKTPLSLNTPPGYVKLTLAGCEERNAQGMCSCAGFTQIVNEARIPACSL

SEQ ID NO: 98 - protein, 410 aa, Artificial Sequence
  APPA-An1
QSEEELKLESVVIVSRHGVRAPTKFTQLMQDVTPYAWPTWPVKLGELTPRGGELIAYLGHYWRQRLVADELLPNQTCPQPGQVAIIADVDERTRKTGEAFAAGLAPGCAITVHHQADTSSPDPLFNPLKTGVCQLDVARVTRAILERAGGSIADFTNHYQPAFRELERVLNFSQSPLCKNREKQNEPCSLTQALPSELKVSADNVSLTGAWSLASMLTEIFLLQQAQGMPEPGWGRITDSHQWNTLLSLHNAYFDLLQRTPEVARSAATPLLDLIKTALTPNGTQKSAYGVTLPTSVLFIAGHDTNLANLGGALELNWTLPGQPDNYPPGGELVFERWRRLSDNSCWIQVSLVFQTLQQMRDKTPLSLNTPPGEVKLTLPGCEERNAQGMCSCAGFTQIVNEARIPACSL

SEQ ID NO: 99 - protein, 410 aa, Artificial Sequence
  APPA-An2
QSEEELKLESVVIVSRHGVRAPTKFTQLMQDVTPYAWPTWPVKLGELTPRGGELIAYLGHYWRQRLVADELLPNQTCPQPGQVAIIADVDERTRKTGEAFAAGLAPGCAITVHHQADTSSPDPLFNPLKTGVCQLDVARVTRAILERAGGSIADFTNHYQPAFRELERVLNFSQSPLCKNREKQNEPCSLTQALPSELKVSADNVSLTGAWSLASMLTEIFLLQQAQGMPEPGWGRITDSHQWNTLLSLHNAYFDLLQRTPEVARSAATPLLDLIKTALTPNGTQKSAYGVTLPTSVLFIAGHDTNLANLGGALELNWTLPGQPDNYPPGGELVFERWRRLSDNSCWIKVSLVFQTLQQMRDKTPLSLNTPPGEVKLTLPGCEERNAQGMCSCAGFTQIVNEARIPACSL

SEQ ID NO: 100 - protein, 410 aa, Artificial Sequence
  APPA-An3
QSEEELKLESVVIVSRHGVRAPTKFTQLMQDVTPYAWPTWPVKLGELTPRGGELIAYLGHYWRQRLVADELLPNQTCPQPGQVAIIADVDERTRKTGEAFAAGLAPGCAITVHHQADTSSPDPLFNPLKTGVCQLDVARVTRAILERAGGSIADFTNHYQPAFRELERVLNFSQSPLCKNREKQNEPCSLTQALPSELKVSADNVSLTGAWSLASMLTEIFLLQQAQGMPEPGWGRITDSHQWNTLLSLHNAYFDLLQRTPEVARSAATPLLDLIKTALTPNGTQKSAYGVTLPTSVLFIAGHDTNLANLGGALELNWTLPGQPDNYPPGGELVFERWRRLSDNSCWIQVSLVFQTLQQMRDKTPLSLNTPPGRVKLTLPGCEERNAQGMCSCAGFTQIVNEARIPACSL

SEQ ID NO: 101 - protein, 410 aa, Artificial Sequence
  APPA-An4
QSEEELKLESVVIVSRHGVRAPTKFTQLMQDVTPYAWPTWPVKLGELTPRGGELIAYLGHYWRQRLVADELLPNQTCPQPGQVAIIADVDERTRKTGEAFAAGLAPGCAITVHHQADTSSPDPLFNPLKTGVCQLDVARVTRAILERAGGSIADFTNHYQPAFRELERVLNFSQSPLCKNREKQNEPCSLTQALPSELKVSADNVSLTGAWSLASMLTEIFLLQQAQGMPEPGWGRITDSHQWNTLLSLHNAYFDLLQRTPEVARSAATPLLDLIKTALTPNGTQKSAYGVTLPTSVLFIAGHDTNLANLGGALELNWTLPGQPDNYPPGGELVFERWRRLSDNSCWIKVSLVFQTLQQMRDKTPLSLNTPPGRVKLTLPGCEERNAQGMCSCAGFTQIVNEARIPACSL

SEQ ID NO: 102 - protein, 410 aa, Artificial Sequence
  APPA-An5
QSEEELKLESVVIVSRHGVRAPTKFTQLMQDVTPYAWPTWPVKLGELTPRGGELIAYLGHYWRQRLVADELLPNQTCPQPGQVAIIADVDERTRKTGEAFAAGLAPDCAITVHHQNDTSSPDPLFNPLKTGVCQLDVARVTRAILERAGGSIADFTNHYQPAFRELERVLNFSQSPLCKNREKQNEPCSLTQALPSELKVSADNVSLTGAWSLASMLTEIFLLQQAQGMPEPGWGRITDSHQWNTLLSLHNAQFDLLQRTPEVARSAATPLLDLIKTALTPNGTQKQAYGVTLPTSVLFIAGHDTNLANLGGALELNWTLPGQPDNYPPGGELVFERWRRLSDNSCWIQVSLVFQTLQQMRDKTPLSLNTPPGEVKLTLPGCEERNAQGMCSCAGFTQIVNEARIPACSL

SEQ ID NO: 103 - protein, 410 aa, Artificial Sequence
  APPA-An6
QSEEELKLESVVIVSRHGVRAPTKFTQLMQDVTPYAWPTWPVKLGELTPRGGELIAYLGHYWRQRLVADELLPNQTCPQPGQVAIIADVDERTRKTGEAFAAGLAPDCAITVHHQNDTSSPDPLFNPLKTGVCQLDVARVTRAILERAGGSIADFTNHYQPAFRELERVLNFSQSPLCKNREKQNEPCSLTQALPSELKVSADNVSLTGAWSLASMLTEIFLLQQAQGMPEPGWGRITDSHQWNTLLSLHNAQFDLLQRTPEVARSAATPLLDLIKTALTPNGTQKQAYGVTLPPSVLFIAGHDTNLANLGGALELNWTLPGQPDNYPPGGELVFERWRRLSDNSCWIQVSLVFQTLQQMRDKTPLSLNTPPGEVKLTLPGCEERNAQGMCSCAGFTQIVNEARIPACSL

SEQ ID NO: 104 - protein, 410 aa, Artificial Sequence
  APPA-An7
QSEEELKLESVVIVSRHGVRAPTKFTQLMQDVTPYAWPTWPVKLGELTPRGGELIAYLGHYWRQRLVADELLPNQTCPQPGQVAIIADVDERTRKTGEAFAAGLAPDCAITVHHQNDTSSPDPLFNPLKTGVCQLDVARVTRAILERAGGSIADFTNHYQPAFRELERVLNFSQSPLCKNREKQNEPCSLTQALPSELKVSADNVSLTGAWSLASMLTEIFLLQQAQGMPEPGWGRITDSHQWNTLLSLHNAQFDLLQRTPEVARSAATPLLDLIKTALTPNGTQKQAYGVTLPTSVLFIAGHDTNLANLGGALELNWTLPGQPDNYPPGGELVFERWRRLSDNSCWIKVSLVFQTLQQMRDKTPLSLNTPPGEVKLTLPGCEERNAQGMCSCAGFTQIVNEARIPACSL

SEQ ID NO: 105 - protein, 410 aa, Artificial Sequence
  APPA-An8
QSEEELKLESVVIVSRHGVRAPTKFTQLMQDVTPYAWPTWPVKLGELTPRGGELIAYLGHYWRQRLVADELLPNQTCPQPGQVAIIADVDERTRKTGEAFAAGLAPDCAITVHHQNDTSSPDPLFNPLKTGVCQLDVARVTRAILERAGGSIADFTNHYQPAFRELERVLNFSQSPLCKNREKQNEPCSLTQALPSELKVSADNVSLTGAWSLASMLTEIFLLQQAQGMPEPGWGRITDSHQWNTLLSLHNAQFDLLQRTPEVARSAATPLLDLIKTALTPNGTQKQAYGVTLPTSVLFIAGHDTNLANLGGALELNWTLPGQPDNYPPGGELVFERWRRLSDNSCWIQVSLVFQTLQQMRDKTPLSLNTPPGRVKLTLPGCEERNAQGMCSCAGFTQIVNEARIPACSL

SEQ ID NO: 106 - protein, 410 aa, Artificial Sequence
  APPA-An9
QSEEELKLESVVIVSRHGVRAPTKFTQLMQDVTPYAWPTWPVKLGELTPRGGELIAYLGHYWRQRLVADELLPNQTCPQPGQVAIIADVDERTRKTGEAFAAGLAPDCAITVHHQNDTSSPDPLFNPLKTGVCQLDVARVTRAILERAGGSIADFTNHYQPAFRELERVLNFSQSPLCKNREKQNEPCSLTQALPSELKVSADNVSLTGAWSLASMLTEIFLLQQAQGMPEPGWGRITDSHQWNTLLSLHNAQFDLLQRTPEVARSAATPLLDLIKTALTPNGTQKQAYGVTLPTSVLFIAGHDTNLANLGGALELNWTLPGQPDNYPPGGELVFERWRRLSDNSCWIKVSLVFQTLQQMRDKTPLSLNTPPGRVKLTLPGCEERNAQGMCSCAGFTQIVNEARIPACSL

SEQ ID NO: 107 - protein, 410 aa, Artificial Sequence
  APPA-An10
QSEEELKLESVVIVSRHGVRAPTKFTQLMQDVTPDAWPTWPVKLGELTPRGGELIAYLGHYWRQRLVADELLPNQTCPQPGQVAIIADVDERTRKTGEAFAAGLAPGCAITVHHQNDTSSPDPLFNPLKTGVCQLDVARVTRAILERAGGSIADFTNHYQPAFRELERVLNFSQSPLCKNREKQNEPCSLTQALPSELKVSADNVSLTGAWSLASMLTEIFLLQQAQGMPEPGWGRITDSHQWNTLLSLHNAYFDLLQRTPEVARSRATPLLDLIKTALTPNGTQKSAYGVTLPTSVLFIAGHDTNLANLGGALELNWTLPGQPDNTPPGGELVFERWRRLSDNSCWIQVSLVFQTLQQMRDKTPLSLNTPPGEVKLTLPGCEERNAQGMCSCAGFTQIVNEARIPACSL

SEQ ID NO: 108 - protein, 410 aa, Artificial Sequence
  APPA-An11
QSEEELKLESVVIVSRHGVRAPTKFTQLMQDVTPDAWPTWPVKLGELTPRGGELIAYLGHYWRQRLVADELLPNQTCPQPGQVAIIADVDERTRKTGEAFAAGLAPGCAITVHHQNDTSSPDPLFNPLKTGVCQLDVARVTRAILERAGGSIADFTNHYQPAFRELERVLNFSQSPLCKNREKQNEPCSLTQALPSELKVSADNVSLTGAWSLASMLTEIFLLQQAQGMPEPGWGRITDSHQWNTLLSLHNAYFDLLQRTPEVARSRATPLLDLIKTALTPNGTQKSAYGVTLPTSVLFIAGHDTNLANLGGALELNWTLPGQPDNTPPGGELVFERWRRLSDNSCWIQVSLVFQTLQQMRDKTPLSLNTPPGRVKLTLPGCEERNAQGMCSCAGFTQIVNEARIPACSL

SEQ ID NO: 109 - protein, 410 aa, Artificial Sequence
  APPA-An12
QSEEELKLESVVIVSRHGVRAPTKFTQLMQDVTPDAWPTWPVKLGELTPRGGELIAYLGHYWRQRLVADELLPNQTCPQPGQVAIIADVDERTRKTGEAFAAGLAPGCAITVHHQNDTSSPDPLFNPLKTGVCQLDVARVTRAILERAGGSIADFTNHYQPAFRELERVLNFSQSPLCKNREKQNEPCSLTQALPSELKVSADNVSLTGAWSLASMLTEIFLLQQAQGMPEPGWGRITDSHQWNTLLSLHNAYFDLLQRTPEVARSRATPLLDLIKTALTPNGTQKSAYGVTLPPSVLFIAGHDTNLANLGGALELNWTLPGQPDNTPPGGELVFERWRRLSDNSCWIKVSLVFQTLQQMRDKTPLSLNTPPGEVKLTLPGCEERNAQGMCSCAGFTQIVNEARIPACSL

SEQ ID NO: 110 - protein, 410 aa, Artificial Sequence
  APPA-An13
QSEEELKLESVVIVSRHGVRAPTKFTQLMQDVTPDAWPTWPVKLGELTPRGGELIAYLGHYWRQRLVADELLPNQTCPQPGQVAIIADVDERTRKTGEAFAAGLAPGCAITVHHQNDTSSPDPLFNPLKTGVCQLDVARVTRAILERAGGSIADFTNHYQPAFRELERVLNFSQSPLCKNREKQNEPCSLTQALPSELKVSADNVSLTGAWSLASMLTEIFLLQQAQGMPEPGWGRITDSHQWNTLLSLHNAYFDLLQRTPEVARSRATPLLDLIKTALTPNGTQKSAYGVTLPPSVLFIAGHDTNLANLGGALELNWTLPGQPDNTPPGGELVFERWRRLSDNSCWIQVSLVFQTLQQMRDKTPLSLNTPPGRVKLTLPGCEERNAQGMCSCAGFTQIVNEARIPACSL

SEQ ID NO: 111 - protein, 410 aa, Artificial Sequence
  APPA-An14
QSEEELKLESVVIVSRHGVRAPTKFTQLMQDVTPDAWPTWPVKLGELTPRGGELIAYLGHYWRQRLVADELLPNQTCPQPGQVAIIADVDERTRKTGEAFAAGLAPGCAITVHHQNDTSSPDPLFNPLKTGVCQLDVARVTRAILERAGGSIADFTNHYQPAFRELERVLNFSQSPLCKNREKQNEPCSLTQALPSELKVSADNVSLTGAWSLASMLTEIFLLQQAQGMPEPGWGRITDSHQWNTLLSLHNAYFDLLQRTPEVARSRATPLLDLIKTALTPNGTQKSAYGVTLPPSVLFIAGHDTNLANLGGALELNWTLPGQPDNTPPGGELVFERWRRLSDNSCWIKVSLVFQTLQQMRDKTPLSLNTPPGRVKLTLPGCEERNAQGMCSCAGFTQIVNEARIPACSL

SEQ ID NO: 112 - protein, 410 aa, Artificial Sequence
  APPA-An15
QSEEELKLESVVIVSRHGVRAPTKFTQLMQDVTPYAWPTWPVKLGELTPRGGELIAYLGHYWRQRLVADELLPNQTCPQPGQVAIIADVDERTRKTGEAFAAGLAPGCAITVHHQADTSSPDPLFNPLKTGVCQLDVARVTRAILERAGGSIADFTNHYQPAFRELERVLNFSQSPLCLNREKQNEPCSLTQALPSELKVSADNVSLTGAWSLASMLTEIFLLQQAEGMPEPGWGRITDSHQWNTLLSLHNAYFDLLQRTPEVARSRATPLLDLIKTALTPNGTQKQAYGVTLPTSVLFIAGHDTNLANLGGALELNWTLPGQPDNYPPGGELVFERWRRLSDNSCWIQVSLVFQTLQQMRDKTPLSLNTPPGEVKLTLPGCEERNAQGMCSCAGFTQIVNEARIPACSL

SEQ ID NO: 113 - protein, 410 aa, Artificial Sequence
  APPA-An16
QSEEELKLESVVIVSRHGVRAPTKFTQLMQDVTPYAWPTWPVKLGELTPRGGELIAYLGHYWRQRLVADELLPNQTCPQPGQVAIIADVDERTRKTGEAFAAGLAPGCAITVHHQADTSSPDPLFNPLKTGVCQLDVARVTRAILERAGGSIADFTNHYQPAFRELERVLNFSQSPLCLNREKQNEPCSLTQALPSELKVSADNVSLTGAWSLASMLTEIFLLQQAEGMPEPGWGRITDSHQWNTLLSLHNAYFDLLQRTPEVARSRATPLLDLIKTALTPNGTQKQAYGVTLPPSVLFIAGHDTNLANLGGALELNWTLPGQPDNYPPGGELVFERWRRLSDNSCWIQVSLVFQTLQQMRDKTPLSLNTPPGEVKLTLPGCEERNAQGMCSCAGFTQIVNEARIPACSL

SEQ ID NO: 114 - protein, 410 aa, Artificial Sequence
  APPA-An17
QSEEELKLESVVIVSRHGVRAPTKFTQLMQDVTPYAWPTWPVKLGELTPRGGELIAYLGHYWRQRLVADELLPNQTCPQPGQVAIIADVDERTRKTGEAFAAGLAPGCAITVHHQADTSSPDPLFNPLKTGVCQLDVARVTRAILERAGGSIADFTNHYQPAFRELERVLNFSQSPLCLNREKQNEPCSLTQALPSELKVSADNVSLTGAWSLASMLTEIFLLQQAEGMPEPGWGRITDSHQWNTLLSLHNAYFDLLQRTPEVARSRATPLLDLIKTALTPNGTQKQAYGVTLPTSVLFIAGHDTNLANLGGALELNWTLPGQPDNYPPGGELVFERWRRLSDNSCWIQVSLVFQTLQQMRDKTPLSLNTPPGRVKLTLPGCEERNAQGMCSCAGFTQIVNEARIPACSL

SEQ ID NO: 115 - protein, 410 aa, Artificial Sequence
  APPA-An18
QSEEELKLESVVIVSRHGVRAPTKFTQLMQDVTPYAWPTWPVKLGELTPRGGELIAYLGHYWRQRLVADELLPNQTCPQPGQVAIIADVDERTRKTGEAFAAGLAPGCAITVHHQADTSSPDPLFNPLKTGVCQLDVARVRRAILERAGGPIADFTNHYQPAFRELERVLNFSQSNLCKKREKQNEPCSLTQALPSELKVSADNVSLTGAWSLASMLTEIFLLQQAQGMPEPGWGRITDSHQWNTLLSLHNAYFDLLQRTPEVARSAATPLLDLIKTALTPNGTQKSAYGVTLPTSVLFIAGHDTNLANLGGALELNWTLPGQPDNYPPGGELVFERWRRLSDNSCWIQVSLVFQTLQQMRDKTPLSLNTPPGEVKLTLPGCEERNAQGMCSCAGFTQIVNEARIPACSL

SEQ ID NO: 116 - protein, 410 aa, Artificial Sequence
  APPA-An19
QSEEELKLESVVIVSRHGVRAPTKFTQLMQDVTPYAWPTWPVKLGELTPRGGELIAYLGHYWRQRLVADELLPNQTCPQPGQVAIIADVDERTRKTGEAFAAGLAPGCAITVHHQADTSSPDPLFNPLKTGVCQLDVARVRRAILERAGGPIADFTNHYQPAFRELERVLNFSQSNLCKKREKQNEPCSLTQALPSELKVSADNVSLTGAWSLASMLTEIFLLQQAQGMPEPGWGRITDSHQWNTLLSLHNAYFDLLQRTPEVARSAATPLLDLIKTALTPNGTQKSAYGVTLPTSVLFIAGHDTNLANLGGALELNWTLPGQPDNYPPGGELVFERWRRLSDNSCWIKVSLVFQTLQQMRDKTPLSLNTPPGEVKLTLPGCEERNAQGMCSCAGFTQIVNEARIPACSL

SEQ ID NO: 117 - protein, 410 aa, Artificial Sequence
  APPA-An20
QSEEELKLESVVIVSRHGVRAPTKFTQLMQDVTPYAWPTWPVKLGELTPRGGELIAYLGHYWRQRLVADELLPNQTCPQPGQVAIIADVDERTRKTGEAFAAGLAPGCAITVHHQADTSSPDPLFNPLKTGVCQLDVARVRRAILERAGGPIADFTNHYQPAFRELERVLNFSQSNLCKKREKQNEPCSLTQALPSELKVSADNVSLTGAWSLASMLTEIFLLQQAQGMPEPGWGRITDSHQWNTLLSLHNAYFDLLQRTPEVARSAATPLLDLIKTALTPNGTQKSAYGVTLPTSVLFIAGHDTNLANLGGALELNWTLPGQPDNYPPGGELVFERWRRLSDNSCWIKVSLVFQTLQQMRDKTPLSLNTPPGRVKLTLPGCEERNAQGMCSCAGFTQIVNEARIPACSL

SEQ ID NO: 118 - protein, 410 aa, Artificial Sequence
  APPA-An21
QSEEELKLESVVIVSRHGVRAPTKFTQLMQDVTPYAWPTWPVKLGELTPRGGELIAYLGHYWRQRLVADELLPNQTCPQPGQVAIIADVDERTRKTGEAFAAGLAPGCAITVHHQADTSSPDPLFNPLKTGVCQLDVARVRRAILERAGGPIADFTNHYQPAFRELERVLNFSQSNLCKKREKQNEPCSLTQALPSELKVSADNVSLTGAWSLASMLTEIFLLQQAQGMPEPGWGRITDSHQWNTLLSLHNAYFDLLQRTPEVARSAATPLLDLIKTALTPNGTQKSAYGVTLPPSVLFIAGHDTNLANLGGALELNWTLPGQPDNYPPGGELVFERWRRLSDNSCWIKVSLVFQTLQQMRDKTPLSLNTPPGRVKLTLPGCEERNAQGMCSCAGFTQIVNEARIPACSL